European Patent Application EP 4 603 151 A1, published August 20, 2025. Title: STABLE COSMETIC COMPOSITION, METHODS AND USES THEREOF. Applicant: SOLFARCOS - SOLUÇÕES FARMACÊUTICAS E COSMÉTICAS, LDA. Application EP. The sequence listing filed with the application follows.

SEQUENCE LISTING (590 sequences)

SEQ ID NO: 1 - protein, 39 aa, synthetic construct
GGVCGPSPPCITTVPGVGVPGVGVPGLGVPGVGVPGVGR

SEQ ID NO: 2 - protein, 43 aa, synthetic construct
GGVCGPSPPCITTVPGVGVPGVGVPGVGVPGVGVPGVGVPGVG

SEQ ID NO: 3 - protein, 43 aa, synthetic construct
GGVCGPSPPCITTGAGAGSGAGAGSGAGAGSGAGAGSGAGAGS

SEQ ID NO: 4 - protein, 28 aa, synthetic construct
GGVCGPSPPCITTGGRPSDSYGAPGGGN

SEQ ID NO: 5 - protein, 43 aa, synthetic construct
GGVCGPSPPCITTGPTGPTGPAGPRGLQGLQGLQGERGEQGPT

SEQ ID NO: 6 - protein, 43 aa, synthetic construct
GGVCGPSPPCITTGGFGGMGGGSGGFGGMGGGSGGFGGMGGGS

SEQ ID NO: 7 - protein, 38 aa, synthetic construct
GGVCGPSPPCITTVPGVGVPGVGVPGLGVPGVGVPGVG

SEQ ID NO: 8 - protein, 13 aa, synthetic construct
GGVCGPSPPCITT

SEQ ID NO: 9 - protein, 10 aa, synthetic construct
GGVCGPSPPC

SEQ ID NO: 10 - protein, 10 aa, synthetic construct
CGPSPPCITT

SEQ ID NO: 11 - protein, 4 aa, synthetic construct
VPGG

SEQ ID NO: 12 - protein, 4 aa, synthetic construct
IPGG

SEQ ID NO: 13 - protein, 5 aa, synthetic construct
VPAVG

SEQ ID NO: 14 - protein, 5 aa, synthetic construct
AVGVP

SEQ ID NO: 15 - protein, 5 aa, synthetic construct
IPGVG

SEQ ID NO: 16 - protein, 5 aa, synthetic construct
LPGVG

SEQ ID NO: 17 - protein, 6 aa, synthetic construct
VAPGVG

SEQ ID NO: 18 - protein, 8 aa, synthetic construct
GVGVPGVG

SEQ ID NO: 19 - protein, 9 aa, synthetic construct
VPGFGVGAG

SEQ ID NO: 20 - protein, 9 aa, synthetic construct
VPGVGVPGG

SEQ ID NO: 21 - protein, 5 aa, synthetic construct
  VARIANT 4: note = Any amino acid
VPGXG

SEQ ID NO: 22 - protein, 23 aa, synthetic construct
GVGVPGVGVPGLGVPGVGVPGVG

SEQ ID NO: 23 - protein, 30 aa, synthetic construct
VPGVGVPGVGVPGVGVPGVGVPGVGVPGVG

SEQ ID NO: 24 - protein, 6 aa, synthetic construct
GAGAGS

SEQ ID NO: 25 - protein, 6 aa, synthetic construct
GAGSGA

SEQ ID NO: 26 - protein, 6 aa, synthetic construct
GAGAGY

SEQ ID NO: 27 - protein, 6 aa, synthetic construct
GAGYGA

SEQ ID NO: 28 - protein, 6 aa, synthetic construct
GAGAGA

SEQ ID NO: 29 - protein, 6 aa, synthetic construct
GAGAGV

SEQ ID NO: 30 - protein, 6 aa, synthetic construct
GAGVGA

SEQ ID NO: 31 - protein, 8 aa, synthetic construct
GAGAGVGY

SEQ ID NO: 32 - protein, 30 aa, synthetic construct
GAGAGSGAGAGSGAGAGSGAGAGSGAGAGS

SEQ ID NO: 33 - protein, 30 aa, synthetic construct
GPTGPTGPAGPRGLQGLQGLQGERGEQGPT

SEQ ID NO: 34 - protein, 15 aa, synthetic construct
GGRPSDSYGAPGGGN

SEQ ID NO: 35 - protein, 11 aa, synthetic construct
GAPAQTPSSQY

SEQ ID NO: 36 - protein, 10 aa, synthetic construct
GGFGGMGGGS

SEQ ID NO: 37 - protein, 4 aa, synthetic construct
MGGG

SEQ ID NO: 38 - protein, 5 aa, synthetic construct
FGGMG

SEQ ID NO: 39 - protein, 7 aa, synthetic construct
FGGMGGG

SEQ ID NO: 40 - protein, 9 aa, synthetic construct
GGFGGMGGG

SEQ ID NO: 41 - protein, 10 aa, synthetic construct
FGGMGGGNAG

SEQ ID NO: 42 - protein, 30 aa, synthetic construct
GGFGGMGGGSGGFGGMGGGSGGFGGMGGGS

SEQ ID NO: 43 - skipped

SEQ ID NO: 44 - protein, 43 aa, synthetic construct
GGVCGPSPPCITTGQGQGQGQGQGQGQGQGQGQGQGQGQGQGQ

SEQ ID NO: 45 - protein, 43 aa, synthetic construct
GGVCGPSPPCITTAKAKAKAKAKAKAKAKAKAKAKAKAKAKAK

SEQ ID NO: 46 - protein, 43 aa, synthetic construct
GGVCGPSPPCITTLKLKLKLKLKLKLKLKLKLKLKLKLKLKLK

SEQ ID NO: 47 - protein, 43 aa, synthetic construct
GGVCGPSPPCITTGAGAGAGAGAGAGAGAGAGAGAGAGAGAGA

SEQ ID NO: 48 - skipped

SEQ ID NO: 49 - protein, 50 aa, synthetic construct
  VARIANT 4: note = Any amino acid
  VARIANT 9: note = Any amino acid
  VARIANT 14: note = Any amino acid
  VARIANT 19: note = Any amino acid
  VARIANT 24: note = Any amino acid
  VARIANT 29: note = Any amino acid
  VARIANT 34: note = Any amino acid
  VARIANT 39: note = Any amino acid
  VARIANT 44: note = Any amino acid
  VARIANT 49: note = Any amino acid
  VARIANT 1..50: note = This sequence may encompass 1-10 VPGXG repeating units
VPGXGVPGXGVPGXGVPGXGVPGXGVPGXGVPGXGVPGXGVPGXGVPGXG

SEQ ID NO: 50 - protein, 5 aa, synthetic construct
VPGVG

SEQ ID NO: 51 - protein, 5 aa, synthetic construct
VPGLG

SEQ ID NO: 52 - protein, 9 aa, synthetic construct
VPGVGVPGL

SEQ ID NO: 53 - protein, 26 aa, synthetic construct
VPGVGVPGVGVPGLGVPGVGVPGVGR

SEQ ID NO: 54 - protein, 25 aa, synthetic construct
VPGVGVPGVGVPGLGVPGVGVPGVG

SEQ ID NO: 55 - protein, 258 aa, synthetic construct
LLNLAGLVPGVGVAPGVGVAPGVGVAPGVGLAPGVGVAPGVGVAPGVGVAPGIGPGGVAAAAKSAAKVAAKAQLRAAAGLGAGIPGLGVGVGVPGLGVGAGVPGLGVGAGVPGFGAVPGALAAAKAAKYGAAVPGVLGGLGALGGVGIPGGVVGAGPAAAAAAAKAAAKAAQFGLVGAAGLGGLGVGGLGVPGVGGLGGIPPAAAAKAAKYGAAGLGGVLGGAGQFPLGGVAARPGFGLSPIFPGGACLGKACGRKRK

SEQ ID NO: 56 - protein, 102 aa, synthetic construct
GYGAGAGSGAASGAGAGSGAGAGSGAGAGSGAGAGSGAGAGSGAGAGSGAGAGSGAGAGYGAGAGVGYGAGAGSGAASGAGAGSGAGAGSGAGAGSGAGAGS

SEQ ID NO: 57 - protein, 6 aa, synthetic construct
GPTGPT

SEQ ID NO: 58 - protein, 6 aa, synthetic construct
GLQGLQ

SEQ ID NO: 59 - protein, 1069 aa, synthetic construct
MFSFVDLRLLLLLAATALLTHGQEEGQVEGQDEDIPPITCVQNGLRYHDRDVWKPEPCRICVCDNGKVLCDDVICDETKNCPGAEVPEGECCPVCPDGSESPTDQETTGVEGPKGDTGPRGPRGPAGPPGRDGIPGQPGLPGPPGPPGPPGPPGLGGNFAPQLSYGYDEKSTGGISVPGPMGPSGPRGLPGPPGAPGPQGFQGPPGEPGEPGASGPMGPRGPPGPPGKNGDDGEAGKPGRPGERGPPGPQGARGLPGTAGLPGMKGHRGFSGLDGAKGDAGPAGPKGEPGSPGENGAPGQMGPRGLPGERGRPGAPGPAGARGNDGATGAAGPPGPTGPAGPPGFPGAVGAKGEAGPQGPRGSEGPQGVRGEPGPPGPAGAAGPAGNPGADGQPGAKGANGAPGIAGAPGFPGARGPSGPQGPGGPPGPKGNSGEPGAPGSKGDTGAKGEPGPVGVQGPPGPAGEEGKRGARGEPGPTGLPGPPGERGGPGSRGFPGADGVAGPKGPAGERGSPGPAGPKGSPGEAGRPGEAGLPGAKGLTGSPGSPGPDGKTGPPGPAGQDGRPGPPGPPGARGQAGVMGFPGPKGAAGEPGKAGERGVPGPPGAVGPAGKDGEAGAQGPPGPAGPAGERGEQGPAGSPGFQGLPGPAGPPGEAGKPGEQGVPGDLGAPGPSGARGERGFPGERGVQGPPGPAGPRGANGAPGNDGAKGDAGAPGAPGSQGAPGLQGMPGERGAAGLPGPKGDRGDAGPKGADGSPGKDGVRGLTGPIGPPGPAGAPGDKGESGPSGPAGPTGARGAPGDRGEPGPPGPAGFAGPPGADGQPGAKGEPGDAGAKGDAGPPGPAGPAGPPGPIGNVGAPGAKGARGSAGPPGATGFPGAAGRVGPPGPSGNAGPPGPPGPAGKEGGKGPRGETGPAGRPGEVGPPGPPGPAGEKGSPGADGPAGAPGTPGPQGIAGQRGVVGLPGQRGERGFPGLPGPSGEPGKQGPSGASGERGPPGPMGPPGLAGPPGESGREGAPGAEGSPGRDGSPGAKGDRGETGPAGPPGAPGAPGAPGPVGPAGKSGDRGET

SEQ ID NO: 60 - protein, 620 aa, synthetic construct
MFKLLGLTLLMAMVVLGRPEPPVNSYLPPSDSYGAPGQSGPGGRPSDSYGAPGGGNGGRPSDSYGAPGQGQGQGQGQGGYAGKPSDTYGAPGGGNGNGGRPSSSYGAPGGGNGGRPSDTYGAPGGGNGGRPSDTYGAPGGGGNGNGGRPSSSYGAPGQGQGNGNGGRSSSSYGAPGGGNGGRPSDTYGAPGGGNGGRPSDTYGAPGGGNNGGRPSSSYGAPGGGNGGRPSDTYGAPGGGNGNGSGGRPSSSYGAPGQGQGGFGGRPSDSYGAPGQNQKPSDSYGAPGSGNGNGGRPSSSYGAPGSGPGGRPSDSYGPPASGSGAGGAGGSGPGGADYDNDEPAKYEFNYQVEDAPSGLSFGHSEMRDGDFTTGQYNVLLPDGRKQIVEYEADQQGYRPQIRYEGDANDGSGPSGPGGPGGQNLGADGYSSGRPGNGNGNGNGGYSGGRPGGQDLGPSGYSGGRPGGQDLGAGGYSNGKPGGQDLGPGGYSGGRPGGQDLGRDGYSGGRPGGQDLGASGYSNGRPGGNGNGGSDGGRVIIGGRVIGGQDGGDQGYSGGRPGGQDLGRDGYSSGRPGGRPGGNGQDSQDGQGYSSGRPGQGGRNGFGPGGQNGDNDGSGYRY

SEQ ID NO: 61 - protein, 131 aa, synthetic construct
MNAYICLAACLIAAVSAAGYGGGAGSMGGTGGMGGGMNAGGFGGMGGMGGGKGGFGGIGGFGGGMGGGPGGFGGMGGFGGMAAKGGFGGMGSGMGGFGGMGGGNAGFGGMGGGNAGFGGMGGQGGFGGKGY

SEQ ID NO: 62 - protein, 18 aa, synthetic construct
GGVCGPSPPCITTVPGVG

SEQ ID NO: 63 - protein, 19 aa, synthetic construct
GGVCGPSPPCITTGAGAGS

SEQ ID NO: 64 - skipped

SEQ ID NO: 65 - protein, 23 aa, synthetic construct
GGVCGPSPPCITTGGFGGMGGGS

SEQ ID NO: 66 - protein, 7 aa, synthetic construct
CGPSPPC

SEQ ID NO: 67 - protein, 9 aa, synthetic construct
GVCGPSPPC

SEQ ID NO: 68 - protein, 10 aa, synthetic construct
CLPCLPAASC

SEQ ID NO: 69 - protein, 7 aa, synthetic construct
CLPAASC

SEQ ID NO: 70 - protein, 8 aa, synthetic construct
YGGSSGGG

SEQ ID NO: 71 - protein, 5 aa, synthetic construct
FGGGS

SEQ ID NO: 72 - protein, 11 aa, synthetic construct
CCQSSCCKPSC

SEQ ID NO: 73 - protein, 11 aa, synthetic construct
CVSSCCKPQCC

SEQ ID NO: 74 - protein, 10 aa, synthetic construct
PITCRRTCYH

SEQ ID NO: 75 - protein, 10 aa, synthetic construct
DCKLPCNPCA

SEQ ID NO: 76 - protein, 10 aa, synthetic construct
CLPCLPAASC

SEQ ID NO: 77 - protein, 10 aa, synthetic construct
CEPAICEPSC

SEQ ID NO: 78 - protein, 11 aa, synthetic construct
CQCSCCKPYCS

SEQ ID NO: 79 - protein, 11 aa, synthetic construct
FCGFPSCSTSC

SEQ ID NO: 80 - protein, 12 aa, synthetic construct
CTPPSCCQLHHA

SEQ ID NO: 81 - protein, 10 aa, synthetic construct
SCCAPVYCCK

SEQ ID NO: 82 - protein, 5 aa, synthetic construct
IPGLG

SEQ ID NO: 83 - protein, 5 aa, synthetic construct
GYGVP

SEQ ID NO: 84 - protein, 5 aa, synthetic construct
GGGVP

SEQ ID NO: 85 - protein, 10 aa, synthetic construct
IPGVGIPGLG

SEQ ID NO: 86 - protein, 10 aa, synthetic construct
IPGVGVPGLG

SEQ ID NO: 87 - protein, 10 aa, synthetic construct
VPGVGVPGLG

SEQ ID NO: 88 - protein, 10 aa, synthetic construct
VPGVGIPGVG

SEQ ID NO: 89 - protein, 10 aa, synthetic construct
VPGVGIPGLG

SEQ ID NO: 90 - protein, 10 aa, synthetic construct
GYGVPGGGVP

SEQ ID NO: 91 - protein, 10 aa, synthetic construct
IPGVGAVGVP

SEQ ID NO: 92 - protein, 6 aa, synthetic construct
  VARIANT 4: note = Any amino acid
  VARIANT 6: note = Any amino acid
GAGXGX

SEQ ID NO: 93 - protein, 6 aa, synthetic construct
  VARIANT 2: note = Any amino acid
  VARIANT 5: note = Any amino acid
GXPGXP

SEQ ID NO: 94 - protein, 6 aa, synthetic construct
  SITE 2: note = 4-hydroxyproline
  SITE 5: note = 4-hydroxyproline
GXPGXP

SEQ ID NO: 95 - protein, 6 aa, synthetic construct
GPAGPA

SEQ ID NO: 96 - protein, 11 aa, synthetic construct
AQTPSSQYGAP

SEQ ID NO: 97 - protein, 30 aa, synthetic construct
GQGQGQGQGQGQGQGQGQGQGQGQGQGQGQ

SEQ ID NO: 98 - protein, 30 aa, synthetic construct
AKAKAKAKAKAKAKAKAKAKAKAKAKAKAK

SEQ ID NO: 99 - protein, 30 aa, synthetic construct
LKLKLKLKLKLKLKLKLKLKLKLKLKLKLK

SEQ ID NO: 100 - protein, 30 aa, synthetic construct
GAGAGAGAGAGAGAGAGAGAGAGAGAGAGA

SEQ ID NO: 101 - protein, 10 aa, synthetic construct
VSSCCKPQCC

SEQ ID NO: 102 - protein, 7 aa, synthetic construct
CCKPQCC

SEQ ID NO: 103 - protein, 10 aa, synthetic construct
CCQSSCCKPS

SEQ ID NO: 104 - protein, 786 aa, synthetic construct
MAGLTAAAPRPGVLLLLLSILHPSRPGGVPGAIPGGVPGGVFYPGAGLGALGGGALGPGGKPLKPVPGGLAGAGLGAGLGAFPAVTFPGALVPGGVADAAAAYKAAKAGAGLGGVPGVGGLGVSAGAVVPQPGAGVKPGKVPGVGLPGVYPGGVLPGARFPGVGVLPGVPTGAGVKPKAPGVGGAFAGIPGVGPFGGPQPGVPLGYPIKAPKLPGGYGLPYTTGKLPYGYGPGGVAGAAGKAGYPTGTGVGPQAAAAAAAKAAAKFGAGAAGVLPGVGGAGVPGVPGAIPGIGGIAGVGTPAAAAAAAAAAKAAKYGAAAGLVPGGPGFGPGVVGVPGAGVPGVGVPGAGIPVVPGAGIPGAAVPGVVSPEAAAKAAAKAAKYGARPGVGVGGIPTYGVGAGGFPGFGVGVGGIPGVAGVPGVGGVPGVGGVPGVGISPEAQAAAAAKAAKYGAAGAGVLGGLVPGAPGAVPGVPGTGGVPGVGTPAAAAAKAAAKAAQFGLVPGVGVAPGVGVAPGVGVAPGVGLAPGVGVAPGVGVAPGVGVAPGIGPGGVAAAAKSAAKVAAKAQLRAAAGLGAGIPGLGVGVGVPGLGVGAGVPGLGVGAGVPGFGAGADEGVRRSLSPELREGDPSSSQHLPSTPSSPRVPGALAAAKAAKYGAAVPGVLGGLGALGGVGIPGGVVGAGPAAAAAAAKAAAKAAQFGLVGAAGLGGLGVGGLGVPGVGGLGGIPPAAAAKAAKYGAAGLGGVLGGAGQFPLGGVAARPGFGLSPIFPGGACLGKACGRKRK

SEQ ID NO: 105 - protein, 5263 aa, synthetic construct
MRVKTFVILCCALQYVAYTNANINDFDEDYFGSDVTVQSSNTTDEIIRDASGAVIEEQITTKKMQRKNKNHGILGKNEKMIKTFVITTDSDGNESIVEEDVLMKTLSDGTVAQSYVAADAGAYSQSGPYVSNSGYSTHQGYTSDFSTSAAVGAGAGAGAAAGSGAGAGAGYGAASGAGAGAGAGAGAGYGTGAGAGAGAGYGAGAGAGAGAGYGAGAGAGAGAGYGAGAGAGAGAGYGAGAGAGAGAGYGAGAGAGAGAGYGAASGAGAGAGYGQGVGSGAASGAGAGAGAGSAAGSGAGAGAGTGAGAGYGAGAGAGAGAGYGAASGTGAGYGAGAGAGYGGASGAGAGAGAGAGAGAGAGYGTGAGYGAGAGAGAGAGAGAGYGAGAGAGYGAGYGVGAGAGYGAGYGAGAGSGAASGAGSGAGAGSGAGAGSGAGAGSGAGAGSGAGAGSGAGAGSGAGAGSGAGAGSGTGAGSGAGAGYGAGAGAGYGAGAGSGAASGAGAGSGAGAGSGAGAGSGAGAGSGAGAGSGAGAGYGAGAGAGYGAGAGAGYGAGAGVGYGAGAGSGAASGAGAGSGAGAGSGAGAGSGAGAGSGAGAGSGAGAGSGAGAGSGAGAGSGAGAGSGAGVGYGAGVGAGYGAGYGAGAGAGYGAGAGSGAASGAGAGAGAGAGTGSSGFGPYVANGGYSRSDGYEYAWSSDFGTGSGAGAGSGAGAGSGAGAGSGAGAGSGAGAGSGAGAGYGAGVGVGYGAGYGAGAGAGYGAGAGSGAASGAGAGSGAGAGSGAGAGSGAGAGSGAGAGSGAGAGSGAGAGSGAGAGSGAGAGSGAGAGSGAGVGSGAGAGSGAGAGVGYGAGAGVGYGAGAGSGAASGAGAGSGAGAGSGAGAGSGAGAGSGAGAGSGAGAGSGAGAGSGAGAGSGAGAGSGAGVGYGAGVGAGYGAGYGAGAGAGYGAGAGSGAASGAGAGSGAGAGSGAGAGSGAGAGSGAGAGSGAGAGSGAGAGSGAGAGSGAGAGSGAGAGSGAGAGSGAGAGYGAGAGAGYGAGYGAGAGAGYGAGAGSGAASGAGSGAGAGSGAGAGAGSGAGAGSGAGAGSGAGAGSGAGAGSGAGAGSGAGAGYGAGVGAGYGAGYGAGAGAGYGAGAGSGAASGAGAGSGAGAGSGAGAGSGAGAGSGAGAGSGAGAGSGAGAGSGAGVGYGAGYGAGAGAGYGAGAGSGAASGAGAGAGAGAGTGSSGFGPYVAHGGYSGYEYAWSSESDFGTGSGAGAGSGAGAGSGAGAGSGAGAGSGAGYGAGVGAGYGAGYGAGAGAGYGAGAGSGAGSGAGAGSGAGAGSGAGAGSGAGAGSGAGAGSGAGAGSGAGAGSGAGAGSGAGAGYGAGYGAGAGAGYGAGAGSGAGSGAGAGSGAGAGSGAGAGSGAGAGSGAGAGSGAGAGSGAGAGSGAGAGYGAGVGAGYGAGYGAGAGAGYGAGAGSGAGSGAGAGSGAGAGSGAGAGSGAGVGSGAGAGSGAGAGSGAGAGSGAGAGYGAGYGAGAGAGYGAGAGSGAGSGAGAGSGAGAGSGAGAGSGAGAGSGAGAGSGAGAGSGAGAGSGAGVGYGAGVGAGYGAGYGAGAGAGYGAGAGSGAASGAGAGAGAGAGTGSSGFGPYVANGGYSGYEYAWSSESDFGTGSGAGAGSGAGAGSGAGAGSGAGAGSGAGAGYGAGYGAGAGAGYGAGAGSGAGSGAGAGSGAGAGSGAGAGSGAGAGSGAGAGSGAGAGSGAGAGSGAGSGSGAGAGSGAGAGSGAGAGYGAGVGAGYGVGYGAGAGAGYGAGAGSGAASGAGAGAGAGAGTGSSGFGPYVAHGGYSGYEYAWSSESDFGTGSGAGAGSGAGAGSGAGAGSGAGAGSGAGAGSGAGAGSGAGAGYGAGVGAGYGAAYGAGAGAGYGAGAGSGAASGAGAGSGAGAGSGAGAGSGAGAGSGAGAGSGAGAGSGAGAGSGAGAGSGAGAGSGAGAGSGAGAGYGAGAGAGYGAGAGSGAGSGAGAGSGAGAGSGAGAGSGAGAGSGAGAGSGAGSGSGAGAGSGAGAGSGAGAGYGAGVGAGYGAGYGAGAGAGYGAGAGSGAGSGAGAGSGAGAGYGAGAGAGYGAGYGAGAGAGYGAGAGTGAGSGAGAGSGAGAGSGAGAGSGAGAGSGAGAGSGAGAGSGAGSGSGAGAGSGAGAGSGAGAGSGAGAGSGAGAGSGAGAGYGAGAGAGYGAGYGAGAGAGYGAGAGSGAGSGAGAGSGAGAGSGAGAGSGAGAGYGAGYGAGAGSGAASGAGAGAGAGAGTGSSGFGPYVAHGGYSGYEYAWSSESDFGTGSGAGAGSGAGAGAGAGAGSGAGAGYGAGVGAGYGAGYGAGAGAGYGAGAGSGTGSGAGAGSGAGAGYGAGVGAGYGAGAGSGAAFGAGAGAGAGSGAGAGSGAGAGSGAGAGSGAGAGSGAGAGYGAGYGAGVGAGYGAGAGSGAASGAGAGSGAGAGSGAGAGSGAGAGSGAGAGSGAGAGYGAGVGAGYGAGYGAGAGAGYGAGAGSGAASGAGAGSGAGAGAGSGAGAGSGAGAGSGAGAGSGAGSGAGAGSGAGAGSGAGAGYGAGAGSGAASGAGAGAGAGAGTGSSGFGPYVANGGYSGYEYAWSSESDFGTGSGAGAGSGAGAGSGAGAGSGAGAGSGAGAGYGAGVGAGYGAGYGAGAGAGYGAGAGSGAGSGAGAGSGAGAGSGAGAGSGAGAGSGAGAGSGAGAGSGAGAGYGAGAGSGAASGAGAGSGAGAGSGAGAGSGAGAGSGAGAGSGAGAGSGAGAGYGAGVGAGYGVGYGAGAGAGYGAGAGSGAGSGAGAGSGAGAGSGAGAGSGAGAGSGAGSGAGAGSGAGAGSGAGAGSGAGSGAGAGSGAGAGYGVGYGAGAGAGYGAGAGSGAGSGAGAGSGAGAGSGAGAGSGAGSGAGAGSGAGAGSGAGAGSGAGAGYGAGVGAGYGVGYGAGAGAGYGAGAGSGAGSGAGAGSGAGAGSGAGAGSGAGAGSGAGAGSGAGAGSGAGAGSGAGSGAGAGSGAGAGSGAGAGSGAGAGSGAGSGAGAGSGAGAGSGAGAGSGAGAGYGAGVGAGYGVGYGAGVGAGYGAGAGSGAASGAGAGSGAGAGAGSGAGAGSGAGAGSGAGAGSGAGAGSGAGAGSGAGAGYGAGYGAGVGAGYGAGAGVGYGAGAGAGYGAGAGSGAASGAGAGAGSGAGAGTGAGAGSGAGAGYGAGAGSGAASGAGAGAGAGAGTGSSGFGPYVANGGYSGYEYAWSSESDFGTGSGAGAGSGAGAGSGAGAGSGAGAGSGAGAGYGAGVGAGYGAGAGSGAGSGAGAGSGAGAGSGAGAGSGAGAGSGAGAGYGAGAGSGTGSGAGAGSGAGAGSGAGAGSGAGAGSGAGAGSGAGAGSGVGAGYGVGYGAGAGAGYGVGYGAGAGAGYGAGAGSGTGSGAGAGSGAGAGSGAGAGSGAGAGSGAGAGSGAGAGSGAGAGYGAGVGAGYGVGYGAGAGAGYGAGAGSGAGSGAGAGSGAGAGSGAGAGSGAGAGSGAGSGAGAGSGAGAGSGAGAGSGAGSGAGAGSGAGAGYGVGYGAGAGAGYGAGAGSGAGSGAGAGSGAGAGSGAGAGSGAGSGAGAGSGAGAGSGAGAGSGAGAGYGAGVGAGYGVGYGAGAGAGYGAGAGSGAGSGAGAGSGAGAGSGAGAGSGAGAGSGAGAGSGAGAGSGAGAGSGAGSGAGAGSGAGAGSGAGAGSGAGAGYGAGVGAGYGVGYGAGAGAGYGAGAGSGAASGAGAGAGAGAGTGSSGFGPYVANGGYSGYEYAWSSESDFGTGSGAGAGSGAGAGSGAGAGYGAGYGAGVGAGYGAGAGVGYGAGAGAGYGAGAGSGAASGAGAGAGAGAGSGAGAGSGAGAGAGSGAGAGYGAGYGIGVGAGYGAGAGVGYGAGAGAGYGAGAGSGAASGAGAGSGAGAGSGAGAGSGAGAGSGAGAGSGAGAGSGAGAGYGAGYGAGVGAGYGAGAGVGYGAGAGAGYGAGAGSGAASGAGAGAGAGAGAGSGAGAGSGAGAGSGAGAGSGAGAGSGAGAGSGAGAGSGAGAGSGAGAGSGAGAGYGAGVGAGYGAGYGGAGAGYGAGAGSGAASGAGAGSGAGAGSGAGAGSGAGAGSGAGAGSGAGAGYGAGAGSGAASGAGAGAGAGAGTGSSGFGPYVNGGYSGYEYAWSSESDFGTGSGAGAGSGAGAGSGAGAGYGAGVGAGYGAGYGAGAGAGYGAGAGSGAASGAGAGSGAGAGSGAGAGSGAGAGSGAGSGAGAGSGAGAGSGAGAGSGAGAGSGAGAGSGAGAGYGAGVGAGYGAGYGAGAGAGYGAGAGSGAASGAGAGSGAGAGAGSGAGAGSGAGAGSGAGAGSGAGAGSGAGAGSGAGSGAGAGSGAGAGYGAGYGAGVGAGYGAGAGVGYGAGAGAGYGAGAGSGAASGAGAGSGSGAGSGAGAGSGAGAGSGAGAGAGSGAGAGSGAGAGSGAGAGYGAGYGAGAGSGAASGAGAGAGAGAGTGSSGFGPYVANGGYSGYEYAWSSESDFGTGSGAGAGSGAGAGSGAGAGYGAGVGAGYGAGYGAGAGAGYGAGAGSGAGSGAGAGSGAGAGSGAGAGSGAGAGSGAGAGSGAGAGSGAGAGSGAGAGYGAGYGAGAGAGYGAGAGVGYGAGAGAGYGAGAGSGAGSGAGAGSGSGAGAGSGSGAGSGAGAGSGAGAGSGAGAGSGAGAGSGAGAGSGAGAGSGAGAGYGAGYGIGVGAGYGAGAGVGYGAGAGAGYGAGAGSGAASGAGAGSGAGAGSGAGAGSGAGAGSGAGAGSGAGAGSGAGAGSGAGAGSGAGAGSGAGAGYGAGAGVGYGAGAGSGAASGAGAGSGAGAGSGAGAGSGAGAGSGAGAGSGAGAGSGAGAGSGAGSGAGAGSGAGAGYGAGYGAGVGAGYGAGAGYGAGYGVGAGAGYGAGAGSGAGSGAGAGSGAGAGSGAGAGSGAGAGSGAGAGSGAGSGAGAGYGAGAGAGYGAGAGAGYGAGAGSGAASGAGAGAGAGSGAGAGSGAGAGSGAGSGAGAGSGAGAGYGAGAGSGAASGAGAGSGAGAGAGAGAGAGSGAGAGSGAGAGYGAGAGSGAASGAGAGAGAGTGSSGFGPYVANGGYSRREGYEYAWSSKSDFETGSGAASGAGAGAGSGAGAGSGAGAGSGAGAGSGAGAGGSVSYGAGRGYGQGAGSAASSVSSASSRSYDYSRRNVRKNCGIPRRQLVVKFRALPCVNC

SEQ ID NO: 106 - protein, 703 aa, Homo sapiens
MLGTLTPLSSLLLLLLVLVLGCGPRASSGGGAGGAAGYAPVKYIQPMQKGPVGPPFREGKGQYLEMPLPLLPMDLKGEPGPPGKPGPRGPPGPPGFPGKPGMGKPGLHGQPGPAGPPGFSRMGKAGPPGLPGKVGPPGQPGLRGEPGIRGDQGLRGPPGPPGLPGPSGITIPGKPGAQGVPGPPGFQGEPGPQGEPGPPGDRGLKGDNGVGQPGLPGAPGQGGAPGPPGLPGPAGLGKPGLDGLPGAPGDKGESGPPGVPGPRGEPGAVGPKGPPGVDGVGVPGAAGLPGPQGPSGAKGEPGTRGPPGLIGPTGYGMPGLPGPKGDRGPAGVPGLLGDRGEPGEDGEPGEQGPQGLGGPPGLPGSAGLPGRRGPPGPKGEAGPGGPPGVPGIRGDQGPSGLAGKPGVPGERGLPGAHGPPGPTGPKGEPGFTGRPGGPGVAGALGQKGDLGLPGQPGLRGPSGIPGLQGPAGPIGPQGLPGLKGEPGLPGPPGEGRAGEPGTAGPTGPPGVPGSPGITGPPGPPGPPGPPGAPGAFDETGIAGLHLPNGGVEGAVLGKGGKPQFGLGELSAHATPAFTAVLTSPFPASGMPVKFDRTLYNGHSGYNPATGIFTCPVGGVYYFAYHVHVKGTNVWVALYKNNVPATYTYDEYKKGYLDQASGGAVLQLRPNDQVWVQMPSDQANGLYSTEYIHSSFSGFLLCPT

SEQ ID NO: 107 - protein, 620 aa, synthetic construct; identical to SEQ ID NO: 60

SEQ ID NO: 108 - protein, 456 aa, synthetic construct
GGRPSDSYGAPGGGNGGRPSDSYGAPGGGNGGRPSDSYGAPGGGNGGRPSDSYGAPGGGNGGRPSDSYGAPGGGNGGRPSDSYGAPGGGNGGRPSDSYGAPGGGNGGRPSDSYGAPGGGNGGRPSDSYGAPGGGNGGRPSDSYGAPGGGNGQGQGQGQGQGQGQGQGQGQGGVCGPSPPCITTGQGQGQGQGQGQGQGQGQGQVPAVGVPAVGVPAVGVPAVGVPAVGVPAVGVPAVGVPAVGVPAVGVPAVGGQGQGQGQGQGQGQGQGQGQGGVCGPSPPCITTGQGQGQGQGQGQGQGQGQGQGGRPSDSYGAPGGGNGGRPSDSYGAPGGGNGGRPSDSYGAPGGGNGGRPSDSYGAPGGGNGGRPSDSYGAPGGGNGGRPSDSYGAPGGGNGGRPSDSYGAPGGGNGGRPSDSYGAPGGGNGGRPSDSYGAPGGGNGGRPSDSYGAPGGGN

SEQ ID NO: 109-199 - skipped (91 entries)

SEQ ID NO: 200 - protein, 36 aa, synthetic construct
GGVCGPSPPCVPGVGVPGVGVPGLGVPGVGVPGVGR

SEQ ID NO: 201 - protein, 40 aa, synthetic construct
GGVCGPSPPCVPGVGVPGVGVPGVGVPGVGVPGVGVPGVG

SEQ ID NO: 202 - protein, 35 aa, synthetic construct
GGVCGPSPPCVPGVGVPGVGVPGLGVPGVGVPGVG

SEQ ID NO: 203 - protein, 36 aa, synthetic construct
CGPSPPCITTVPGVGVPGVGVPGLGVPGVGVPGVGR

SEQ ID NO: 204 - protein, 40 aa, synthetic construct
CGPSPPCITTVPGVGVPGVGVPGVGVPGVGVPGVGVPGVG

SEQ ID NO: 205 - protein, 35 aa, synthetic construct
CGPSPPCITTVPGVGVPGVGVPGLGVPGVGVPGVG

SEQ ID NO: 206 - protein, 34 aa, synthetic construct
YGGSSGGGVPGVGVPGVGVPGLGVPGVGVPGVGR

SEQ ID NO: 207 - protein, 38 aa, synthetic construct
YGGSSGGGVPGVGVPGVGVPGVGVPGVGVPGVGVPGVG

SEQ ID NO: 208 - protein, 33 aa, synthetic construct
YGGSSGGGVPGVGVPGVGVPGLGVPGVGVPGVG

SEQ ID NO: 209 - protein, 31 aa, synthetic construct
FGGGSVPGVGVPGVGVPGLGVPGVGVPGVGR

SEQ ID NO: 210 - protein, 35 aa, synthetic construct
FGGGSVPGVGVPGVGVPGVGVPGVGVPGVGVPGVG

SEQ ID NO: 211 - protein, 30 aa, synthetic construct
FGGGSVPGVGVPGVGVPGLGVPGVGVPGVG

SEQ ID NO: 212 - protein, 37 aa, synthetic construct
CCQSSCCKPSCVPGVGVPGVGVPGLGVPGVGVPGVGR

SEQ ID NO: 213 - protein, 41 aa, synthetic construct
CCQSSCCKPSCVPGVGVPGVGVPGVGVPGVGVPGVGVPGVG

SEQ ID NO: 214 - protein, 36 aa, synthetic construct
CCQSSCCKPSCVPGVGVPGVGVPGLGVPGVGVPGVG

SEQ ID NO: 215 - protein, 37 aa, synthetic construct
CVSSCCKPQCCVPGVGVPGVGVPGLGVPGVGVPGVGR

SEQ ID NO: 216 - protein, 41 aa, synthetic construct
CVSSCCKPQCCVPGVGVPGVGVPGVGVPGVGVPGVGVPGVG

SEQ ID NO: 217 - protein, 36 aa, synthetic construct
CVSSCCKPQCCVPGVGVPGVGVPGLGVPGVGVPGVG

SEQ ID NO: 218 - protein, 36 aa, synthetic construct
PITCRRTCYHVPGVGVPGVGVPGLGVPGVGVPGVGR

SEQ ID NO: 219 - protein, 40 aa, synthetic construct
PITCRRTCYHVPGVGVPGVGVPGVGVPGVGVPGVGVPGVG

SEQ ID NO: 220 - protein, 35 aa, synthetic construct
PITCRRTCYHVPGVGVPGVGVPGLGVPGVGVPGVG

SEQ ID NO: 221 - protein, 36 aa, synthetic construct
DCKLPCNPCAVPGVGVPGVGVPGLGVPGVGVPGVGR

SEQ ID NO: 222 - protein, 40 aa, synthetic construct
DCKLPCNPCAVPGVGVPGVGVPGVGVPGVGVPGVGVPGVG

SEQ ID NO: 223 - protein, 35 aa, synthetic construct
DCKLPCNPCAVPGVGVPGVGVPGLGVPGVGVPGVG

SEQ ID NO: 224 - protein, 36 aa, synthetic construct
CLPCLPAASCVPGVGVPGVGVPGLGVPGVGVPGVGR

SEQ ID NO: 225 - protein, 40 aa, synthetic construct
CLPCLPAASCVPGVGVPGVGVPGVGVPGVGVPGVGVPGVG

SEQ ID NO: 226 - protein, 35 aa, synthetic construct
CLPCLPAASCVPGVGVPGVGVPGLGVPGVGVPGVG

SEQ ID NO: 227 - protein, 36 aa, synthetic construct
CEPAICEPSCVPGVGVPGVGVPGLGVPGVGVPGVGR

SEQ ID NO: 228 - protein, 40 aa, synthetic construct
CEPAICEPSCVPGVGVPGVGVPGVGVPGVGVPGVGVPGVG

SEQ ID NO: 229 - protein, 35 aa, synthetic construct
CEPAICEPSCVPGVGVPGVGVPGLGVPGVGVPGVG

SEQ ID NO: 230 - protein, 37 aa, synthetic construct
CQCSCCKPYCSVPGVGVPGVGVPGLGVPGVGVPGVGR

SEQ ID NO: 231 - protein, 41 aa, synthetic construct
CQCSCCKPYCSVPGVGVPGVGVPGVGVPGVGVPGVGVPGVG

SEQ ID NO: 232 - protein, 36 aa, synthetic construct
CQCSCCKPYCSVPGVGVPGVGVPGLGVPGVGVPGVG

SEQ ID NO: 233 - protein, 37 aa, synthetic construct
FCGFPSCSTSCVPGVGVPGVGVPGLGVPGVGVPGVGR

SEQ ID NO: 234 - protein, 41 aa, synthetic construct
FCGFPSCSTSCVPGVGVPGVGVPGVGVPGVGVPGVGVPGVG

SEQ ID NO: 235 - protein, 36 aa, synthetic construct
FCGFPSCSTSCVPGVGVPGVGVPGLGVPGVGVPGVG

SEQ ID NO: 236 - protein, 38 aa, synthetic construct
CTPPSCCQLHHAVPGVGVPGVGVPGLGVPGVGVPGVGR

SEQ ID NO: 237 - protein, 42 aa, synthetic construct
CTPPSCCQLHHAVPGVGVPGVGVPGVGVPGVGVPGVGVPGVG

SEQ ID NO: 238 - protein, 37 aa, synthetic construct
CTPPSCCQLHHAVPGVGVPGVGVPGLGVPGVGVPGVG

SEQ ID NO: 239 - protein, 36 aa, synthetic construct
SCCAPVYCCKVPGVGVPGVGVPGLGVPGVGVPGVGR

SEQ ID NO: 240 - protein, 40 aa, synthetic construct
SCCAPVYCCKVPGVGVPGVGVPGVGVPGVGVPGVGVPGVG

SEQ ID NO: 241 - protein, 35 aa, synthetic construct
SCCAPVYCCKVPGVGVPGVGVPGLGVPGVGVPGVG

SEQ ID NO: 242 - protein, 36 aa, synthetic construct
  VARIANT 14..36: note = This region may encompass one of the following sequences: VPGG or IPGG or VPAVG or AVGVP or IPGVG or LPGVG or VAPGVG or GVGVPGVG or VPGFGVGAG or VPGVGVPGG or GVGVPGVGVPGLGVPGVGVPGVG or VPGVG or VPGLG or VPGVGVPGL or IPGLG or GYGVP or GGGVP or IPGVGIPGLG or IPGVGVPGLG or VPGVGVPGLG or VPGVGIPGVG or VPGVGIPGLG or GYGVPGGGVP or IPGVGAVGVP
GGVCGPSPPCITTXXXXXXXXXXXXXXXXXXXXXXX

SEQ ID NO: 243 - protein, 33 aa, synthetic construct
  VARIANT 11..33: note = This region may encompass one of the following sequences: VPGG or IPGG or VPAVG or AVGVP or IPGVG or LPGVG or VAPGVG or GVGVPGVG or VPGFGVGAG or VPGVGVPGG or GVGVPGVGVPGLGVPGVGVPGVG or VPGVG or VPGLG or VPGVGVPGL or IPGLG or GYGVP or GGGVP or IPGVGIPGLG or IPGVGVPGLG or VPGVGVPGLG or VPGVGIPGVG or VPGVGIPGLG or GYGVPGGGVP or IPGVGAVGVP
GGVCGPSPPCXXXXXXXXXXXXXXXXXXXXXXX

SEQ ID NO: 244 - protein, 33 aa, synthetic construct
  VARIANT 11..33: note = This region may encompass one of the following sequences: VPGG or IPGG or VPAVG or AVGVP or IPGVG or LPGVG or VAPGVG or GVGVPGVG or VPGFGVGAG or VPGVGVPGG or GVGVPGVGVPGLGVPGVGVPGVG or VPGVG or VPGLG or VPGVGVPGL or IPGLG or GYGVP or GGGVP or IPGVGIPGLG or IPGVGVPGLG or VPGVGVPGLG or VPGVGIPGVG or VPGVGIPGLG or GYGVPGGGVP or IPGVGAVGVP
CGPSPPCITTXXXXXXXXXXXXXXXXXXXXXXX

SEQ ID NO: 245 - protein, 31 aa, synthetic construct
  VARIANT 9..31: note = This region may encompass one of the following sequences: VPGG or IPGG or VPAVG or AVGVP or IPGVG or LPGVG or VAPGVG or GVGVPGVG or VPGFGVGAG or VPGVGVPGG or GVGVPGVGVPGLGVPGVGVPGVG or VPGVG or VPGLG or VPGVGVPGL or IPGLG or GYGVP or GGGVP or IPGVGIPGLG or IPGVGVPGLG or VPGVGVPGLG or VPGVGIPGVG or VPGVGIPGLG or GYGVPGGGVP or IPGVGAVGVP
YGGSSGGGXXXXXXXXXXXXXXXXXXXXXXX

SEQ ID NO: 246 - protein, 28 aa, synthetic construct
  VARIANT 6..28: note = This region may encompass one of the following sequences: VPGG or IPGG or VPAVG or AVGVP or IPGVG or LPGVG or VAPGVG or GVGVPGVG or VPGFGVGAG or VPGVGVPGG or GVGVPGVGVPGLGVPGVGVPGVG or VPGVG or VPGLG or VPGVGVPGL or IPGLG or GYGVP or GGGVP or IPGVGIPGLG or IPGVGVPGLG or VPGVGVPGLG or VPGVGIPGVG or VPGVGIPGLG or GYGVPGGGVP or IPGVGAVGVP
FGGGSXXXXXXXXXXXXXXXXXXXXXXX

SEQ ID NO: 247 - protein, 34 aa, synthetic construct
  VARIANT 12..34: note = This region may encompass one of the following sequences: VPGG or IPGG or VPAVG or AVGVP or IPGVG or LPGVG or VAPGVG or GVGVPGVG or VPGFGVGAG or VPGVGVPGG or GVGVPGVGVPGLGVPGVGVPGVG or VPGVG or VPGLG or VPGVGVPGL or IPGLG or GYGVP or GGGVP or IPGVGIPGLG or IPGVGVPGLG or VPGVGVPGLG or VPGVGIPGVG or VPGVGIPGLG or GYGVPGGGVP or IPGVGAVGVP
CCQSSCCKPSCXXXXXXXXXXXXXXXXXXXXXXX

SEQ ID NO: 248 - protein, 34 aa, synthetic construct
  VARIANT 12..34: note = This region may encompass one of the following sequences: VPGG or IPGG or VPAVG or AVGVP or IPGVG or LPGVG or VAPGVG or GVGVPGVG or VPGFGVGAG or VPGVGVPGG or GVGVPGVGVPGLGVPGVGVPGVG or VPGVG or VPGLG or VPGVGVPGL or IPGLG or GYGVP or GGGVP or IPGVGIPGLG or IPGVGVPGLG or VPGVGVPGLG or VPGVGIPGVG or VPGVGIPGLG or GYGVPGGGVP or IPGVGAVGVP
CVSSCCKPQCCXXXXXXXXXXXXXXXXXXXXXXX

SEQ ID NO: 249 - protein, 33 aa, synthetic construct
  VARIANT 11..33: note = This region may encompass one of the following sequences: VPGG or IPGG or VPAVG or AVGVP or IPGVG or LPGVG or VAPGVG or GVGVPGVG or VPGFGVGAG or VPGVGVPGG or GVGVPGVGVPGLGVPGVGVPGVG or VPGVG or VPGLG or VPGVGVPGL or IPGLG or GYGVP or GGGVP or IPGVGIPGLG or IPGVGVPGLG or VPGVGVPGLG or VPGVGIPGVG or VPGVGIPGLG or GYGVPGGGVP or IPGVGAVGVP
PITCRRTCYHXXXXXXXXXXXXXXXXXXXXXXX

SEQ ID NO: 250 - protein, 33 aa, synthetic construct
  VARIANT 11..33: note = This region may encompass one of the following sequences: VPGG or IPGG or VPAVG or AVGVP or IPGVG or LPGVG or VAPGVG or GVGVPGVG or VPGFGVGAG or VPGVGVPGG or GVGVPGVGVPGLGVPGVGVPGVG or VPGVG or VPGLG or VPGVGVPGL or IPGLG or GYGVP or GGGVP or IPGVGIPGLG or IPGVGVPGLG or VPGVGVPGLG or VPGVGIPGVG or VPGVGIPGLG or GYGVPGGGVP or IPGVGAVGVP
DCKLPCNPCAXXXXXXXXXXXXXXXXXXXXXXX

SEQ ID NO: 251 - protein, 33 aa, synthetic construct
  VARIANT 11..33: note = This region may encompass one of the following sequences: VPGG or IPGG or VPAVG or AVGVP or IPGVG or LPGVG or VAPGVG or GVGVPGVG or VPGFGVGAG or VPGVGVPGG or GVGVPGVGVPGLGVPGVGVPGVG or VPGVG or VPGLG or VPGVGVPGL or IPGLG or GYGVP or GGGVP or IPGVGIPGLG or IPGVGVPGLG or VPGVGVPGLG or VPGVGIPGVG or VPGVGIPGLG or GYGVPGGGVP or IPGVGAVGVP
CLPCLPAASCXXXXXXXXXXXXXXXXXXXXXXX

SEQ ID NO: 252 - protein, 33 aa, synthetic construct
  VARIANT 11..33: note = This region may encompass one of the following sequences: VPGG or IPGG or VPAVG or AVGVP or IPGVG or LPGVG or VAPGVG or GVGVPGVG or VPGFGVGAG or VPGVGVPGG or GVGVPGVGVPGLGVPGVGVPGVG or VPGVG or VPGLG or VPGVGVPGL or IPGLG or GYGVP or GGGVP or IPGVGIPGLG or IPGVGVPGLG or VPGVGVPGLG or VPGVGIPGVG or VPGVGIPGLG or GYGVPGGGVP or IPGVGAVGVP
CEPAICEPSCXXXXXXXXXXXXXXXXXXXXXXX

SEQ ID NO: 253 - protein, 34 aa, synthetic construct
  VARIANT 12..34: note = This region may encompass one of the following sequences: VPGG or IPGG or VPAVG or AVGVP or IPGVG or LPGVG or VAPGVG or GVGVPGVG or VPGFGVGAG or VPGVGVPGG or GVGVPGVGVPGLGVPGVGVPGVG or VPGVG or VPGLG or VPGVGVPGL or IPGLG or GYGVP or GGGVP or IPGVGIPGLG or IPGVGVPGLG or VPGVGVPGLG or VPGVGIPGVG or VPGVGIPGLG or GYGVPGGGVP or IPGVGAVGVP
CQCSCCKPYCSXXXXXXXXXXXXXXXXXXXXXXX

SEQ ID NO: 254 - protein, 34 aa, synthetic construct
  VARIANT 12..34: note = This region may encompass one of the following sequences: VPGG or IPGG or VPAVG or AVGVP or IPGVG or LPGVG or VAPGVG or GVGVPGVG or VPGFGVGAG or VPGVGVPGG or GVGVPGVGVPGLGVPGVGVPGVG or VPGVG or VPGLG or VPGVGVPGL or IPGLG or GYGVP or GGGVP or IPGVGIPGLG or IPGVGVPGLG or VPGVGVPGLG or VPGVGIPGVG or VPGVGIPGLG or GYGVPGGGVP or IPGVGAVGVP
FCGFPSCSTSCXXXXXXXXXXXXXXXXXXXXXXX

SEQ ID NO: 255 - protein, 35 aa, synthetic construct
  VARIANT 13..35: note = This region may encompass one of the following sequences: VPGG or IPGG or VPAVG or AVGVP or IPGVG or LPGVG or VAPGVG or GVGVPGVG or VPGFGVGAG or VPGVGVPGG or GVGVPGVGVPGLGVPGVGVPGVG or VPGVG or VPGLG or VPGVGVPGL or IPGLG or GYGVP or GGGVP or IPGVGIPGLG or IPGVGVPGLG or VPGVGVPGLG or VPGVGIPGVG or VPGVGIPGLG or GYGVPGGGVP or IPGVGAVGVP
CTPPSCCQLHHAXXXXXXXXXXXXXXXXXXXXXXX

SEQ ID NO: 256 - protein, 33 aa, synthetic construct
  VARIANT 11..33: note = This region may encompass one of the following sequences: VPGG or IPGG or VPAVG or AVGVP or IPGVG or LPGVG or VAPGVG or GVGVPGVG or VPGFGVGAG or VPGVGVPGG or GVGVPGVGVPGLGVPGVGVPGVG or VPGVG or VPGLG or VPGVGVPGL or IPGLG or GYGVP or GGGVP or IPGVGIPGLG or IPGVGVPGLG or VPGVGVPGLG or VPGVGIPGVG or VPGVGIPGLG or GYGVPGGGVP or IPGVGAVGVP
SCCAPVYCCKXXXXXXXXXXXXXXXXXXXXXXX

SEQ ID NO: 257 - protein, 63 aa, synthetic construct
  VARIANT 17: note = Any amino acid
  VARIANT 22: note = Any amino acid
  VARIANT 27: note = Any amino acid
  VARIANT 32: note = Any amino acid
  VARIANT 37: note = Any amino acid
  VARIANT 42: note = Any amino acid
  VARIANT 47: note = Any amino acid
  VARIANT 52: note = Any amino acid
  VARIANT 57: note = Any amino acid
  VARIANT 62: note = Any amino acid
  VARIANT 14..63: note = This region may encompass 1-10 VPGXG repeating units
GGVCGPSPPCITTVPGXGVPGXGVPGXGVPGXGVPGXGVPGXGVPGXGVPGXGVPGXGVPGXG

SEQ ID NO: 258 - protein, 60 aa, synthetic construct
  VARIANT 14: note = Any amino acid
  VARIANT 19: note = Any amino acid
  VARIANT 24: note = Any amino acid
  VARIANT 29: note = Any amino acid
  VARIANT 34: note = Any amino acid
  VARIANT 39: note = Any amino acid
  VARIANT 44: note = Any amino acid
  VARIANT 49: note = Any amino acid
  VARIANT 54: note = Any amino acid
  VARIANT 59: note = Any amino acid
  VARIANT 11..60: note = This region may encompass 1-10 VPGXG repeating units
GGVCGPSPPCVPGXGVPGXGVPGXGVPGXGVPGXGVPGXGVPGXGVPGXGVPGXGVPGXG

SEQ ID NO: 259 - protein, 60 aa, synthetic construct
  VARIANT 14: note = Any amino acid
  VARIANT 19: note = Any amino acid
  VARIANT 24: note = Any amino acid
  VARIANT 29: note = Any amino acid
  VARIANT 34: note = Any amino acid
  VARIANT 39: note = Any amino acid
  VARIANT 44: note = Any amino acid
  VARIANT 49: note = Any amino acid
  VARIANT 54: note = Any amino acid
  VARIANT 59: note = Any amino acid
  VARIANT 11..60: note = This region may encompass 1-10 VPGXG repeating units
CGPSPPCITTVPGXGVPGXGVPGXGVPGXGVPGXGVPGXGVPGXGVPGXGVPGXGVPGXG

SEQ ID NO: 260 - protein, 58 aa, synthetic construct
  VARIANT 12: note = Any amino acid
  VARIANT 17: note = Any amino acid
  VARIANT 22: note = Any amino acid
  VARIANT 27: note = Any amino acid
  VARIANT 32: note = Any amino acid
  VARIANT 37: note = Any amino acid
  VARIANT 42: note = Any amino acid
  VARIANT 47: note = Any amino acid
  VARIANT 52: note = Any amino acid
  VARIANT 57: note = Any amino acid
  VARIANT 9..58: note = This region may encompass 1-10 VPGXG repeating units
YGGSSGGGVPGXGVPGXGVPGXGVPGXGVPGXGVPGXGVPGXGVPGXGVPGXGVPGXG

SEQ ID NO: 261 - protein, 55 aa, synthetic construct
  VARIANT 9: note = Any amino acid
  VARIANT 14: note = Any amino acid
  VARIANT 19: note = Any amino acid
  VARIANT 24: note = Any amino acid
  VARIANT 29: note = Any amino acid
  VARIANT 34: note = Any amino acid
  VARIANT 39: note = Any amino acid
  VARIANT 44: note = Any amino acid
  VARIANT 49: note = Any amino acid
  VARIANT 54: note = Any amino acid
  VARIANT 6..55: note = This region may encompass 1-10 VPGXG repeating units
FGGGSVPGXGVPGXGVPGXGVPGXGVPGXGVPGXGVPGXGVPGXGVPGXGVPGXG

SEQ ID NO: 262 - protein, 61 aa, synthetic construct
  VARIANT 15: note = Any amino acid
  VARIANT 20: note = Any amino acid
  VARIANT 25: note = Any amino acid
  VARIANT 30: note = Any amino acid
  VARIANT 35: note = Any amino acid
  VARIANT 40: note = Any amino acid
  VARIANT 45: note = Any amino acid
  VARIANT 50: note = Any amino acid
  VARIANT 55: note = Any amino acid
  VARIANT 60: note = Any amino acid
  VARIANT 12..61: note = This region may encompass 1-10 VPGXG repeating units
CCQSSCCKPSCVPGXGVPGXGVPGXGVPGXGVPGXGVPGXGVPGXGVPGXGVPGXGVPGXG

SEQ ID NO: 263 - protein, 61 aa, synthetic construct
  VARIANT 15: note = Any amino acid
  VARIANT 20: note = Any amino acid
  VARIANT 25: note = Any amino acid
  VARIANT 30: note = Any amino acid
  VARIANT 35: note = Any amino acid
  VARIANT 40: note = Any amino acid
  VARIANT 45: note = Any amino acid
  VARIANT 50: note = Any amino acid
  VARIANT 55: note = Any amino acid
  VARIANT 60: note = Any amino acid
  VARIANT 12..61: note = This region may encompass 1-10 VPGXG repeating units
CVSSCCKPQCCVPGXGVPGXGVPGXGVPGXGVPGXGVPGXGVPGXGVPGXGVPGXGVPGXG

SEQ ID NO: 264 - protein, 60 aa, synthetic construct
  VARIANT 14: note = Any amino acid
  VARIANT 19: note = Any amino acid
  VARIANT 24: note = Any amino acid
  VARIANT 29: note = Any amino acid
  VARIANT 34: note = Any amino acid
  VARIANT 39: note = Any amino acid
  VARIANT 44: note = Any amino acid
  VARIANT 49: note = Any amino acid
  VARIANT 54: note = Any amino acid
  VARIANT 59: note = Any amino acid
  VARIANT 11..60: note = This region may encompass 1-10 VPGXG repeating units
PITCRRTCYHVPGXGVPGXGVPGXGVPGXGVPGXGVPGXGVPGXGVPGXGVPGXGVPGXG

SEQ ID NO: 265 - protein, 60 aa, synthetic construct
  VARIANT 14: note = Any amino acid
  VARIANT 19: note = Any amino acid
  VARIANT 24: note = Any amino acid
  VARIANT 29: note = Any amino acid
  VARIANT 34: note = Any amino acid
  VARIANT 39: note = Any amino acid
  VARIANT 44: note = Any amino acid
  VARIANT 49: note = Any amino acid
  VARIANT 54: note = Any amino acid
  VARIANT 59: note = Any amino acid
  VARIANT 11..60: note = This region may encompass 1-10 VPGXG repeating units
DCKLPCNPCAVPGXGVPGXGVPGXGVPGXGVPGXGVPGXGVPGXGVPGXGVPGXGVPGXG

SEQ ID NO: 266 - protein, 60 aa, synthetic construct
  VARIANT 14: note = Any amino acid
  VARIANT 19: note = Any amino acid
  VARIANT 24: note = Any amino acid
  VARIANT 29: note = Any amino acid
  VARIANT 34: note = Any amino acid
  VARIANT 39: note = Any amino acid
  VARIANT 44: note = Any amino acid
  VARIANT 49: note = Any amino acid
  VARIANT 54: note = Any amino acid
  VARIANT 59: note = Any amino acid
  VARIANT 11..60: note = This region may encompass 1-10 VPGXG repeating units
CLPCLPAASCVPGXGVPGXGVPGXGVPGXGVPGXGVPGXGVPGXGVPGXGVPGXGVPGXG

SEQ ID NO: 267 - protein, 60 aa, synthetic construct
  VARIANT 14: note = Any amino acid
  VARIANT 19: note = Any amino acid
  VARIANT 24: note = Any amino acid
  VARIANT 29: note = Any amino acid
  VARIANT 34: note = Any amino acid
  VARIANT 39: note = Any amino acid
  VARIANT 44: note = Any amino acid
  VARIANT 49: note = Any amino acid
  VARIANT 54: note = Any amino acid
  VARIANT 59: note = Any amino acid
  VARIANT 11..60: note = This region may encompass 1-10 VPGXG repeating units
CEPAICEPSCVPGXGVPGXGVPGXGVPGXGVPGXGVPGXGVPGXGVPGXGVPGXGVPGXG

SEQ ID NO: 268 - protein, 61 aa, synthetic construct
  VARIANT 15: note = Any amino acid
  VARIANT 20: note = Any amino acid
  VARIANT 25: note = Any amino acid
  VARIANT 30: note = Any amino acid
  VARIANT 35: note = Any amino acid
  VARIANT 40: note = Any amino acid
  VARIANT 45: note = Any amino acid
  VARIANT 50: note = Any amino acid
  VARIANT 55: note = Any amino acid
  VARIANT 60: note = Any amino acid
  VARIANT 12..61: note = This region may encompass 1-10 VPGXG repeating units
CQCSCCKPYCSVPGXGVPGXGVPGXGVPGXGVPGXGVPGXGVPGXGVPGXGVPGXGVPGXG

SEQ ID NO: 269 - protein, 61 aa, synthetic construct
  VARIANT 15: note = Any amino acid
  VARIANT 20: note = Any amino acid
  VARIANT 25: note = Any amino acid
  VARIANT 30: note = Any amino acid
  VARIANT 35: note = Any amino acid
  VARIANT 40: note = Any amino acid
  VARIANT 45: note = Any amino acid
  VARIANT 50: note = Any amino acid
  VARIANT 55: note = Any amino acid
  VARIANT 60: note = Any amino acid
  VARIANT 12..61: note = This region may encompass 1-10 VPGXG repeating units
FCGFPSCSTSCVPGXGVPGXGVPGXGVPGXGVPGXGVPGXGVPGXGVPGXGVPGXGVPGXG

SEQ ID NO: 270 - protein, 62 aa, synthetic construct
  VARIANT 16: note = Any amino acid
  VARIANT 21: note = Any amino acid
  VARIANT 26: note = Any amino acid
  VARIANT 31: note = Any amino acid
  VARIANT 36: note = Any amino acid
  VARIANT 41: note = Any amino acid
  VARIANT 46: note = Any amino acid
  VARIANT 51: note = Any amino acid
  VARIANT 56: note = Any amino acid
  VARIANT 61: note = Any amino acid
  VARIANT 13..62: note = This region may encompass 1-10 VPGXG repeating units
CTPPSCCQLHHAVPGXGVPGXGVPGXGVPGXGVPGXGVPGXGVPGXGVPGXGVPGXGVPGXG

SEQ ID NO: 271 - protein, 60 aa, synthetic construct
  VARIANT 14: note = Any amino acid
  VARIANT 19: note = Any amino acid
  VARIANT 24: note = Any amino acid
  VARIANT 29: note = Any amino acid
  VARIANT 34: note = Any amino acid
  VARIANT 39: note = Any amino acid
  VARIANT 44: note = Any amino acid
  VARIANT 49: note = Any amino acid
  VARIANT 54: note = Any amino acid
  VARIANT 59: note = Any amino acid
  VARIANT 11..60: note = This region may encompass 1-10 VPGXG repeating units
SCCAPVYCCKVPGXGVPGXGVPGXGVPGXGVPGXGVPGXGVPGXGVPGXGVPGXGVPGXG

SEQ ID NO: 272 - protein, 40 aa, synthetic construct
GGVCGPSPPCGAGAGSGAGAGSGAGAGSGAGAGSGAGAGS

SEQ ID NO: 273 - protein, 40 aa, synthetic construct
CGPSPPCITTGAGAGSGAGAGSGAGAGSGAGAGSGAGAGS

SEQ ID NO: 274 - protein, 38 aa, synthetic construct
YGGSSGGGGAGAGSGAGAGSGAGAGSGAGAGSGAGAGS

SEQ ID NO: 275 - protein, 35 aa, synthetic construct
FGGGSGAGAGSGAGAGSGAGAGSGAGAGSGAGAGS

SEQ ID NO: 276 - protein, 41 aa, synthetic construct
CCQSSCCKPSCGAGAGSGAGAGSGAGAGSGAGAGSGAGAGS

SEQ ID NO: 277 - protein, 41 aa, synthetic construct
CVSSCCKPQCCGAGAGSGAGAGSGAGAGSGAGAGSGAGAGS

SEQ ID NO: 278 - protein, 40 aa, synthetic construct
PITCRRTCYHGAGAGSGAGAGSGAGAGSGAGAGSGAGAGS

SEQ ID NO: 279 - protein, 40 aa, synthetic construct
DCKLPCNPCAGAGAGSGAGAGSGAGAGSGAGAGSGAGAGS

SEQ ID NO: 280 - protein, 40 aa, synthetic construct
CLPCLPAASCGAGAGSGAGAGSGAGAGSGAGAGSGAGAGS

SEQ ID NO: 281 - protein, 40 aa, synthetic construct
CEPAICEPSCGAGAGSGAGAGSGAGAGSGAGAGSGAGAGS

SEQ ID NO: 282 - protein, 41 aa, synthetic construct
CQCSCCKPYCSGAGAGSGAGAGSGAGAGSGAGAGSGAGAGS

SEQ ID NO: 283 - protein, 41 aa, synthetic construct
FCGFPSCSTSCGAGAGSGAGAGSGAGAGSGAGAGSGAGAGS

SEQ ID NO: 284 - protein, 42 aa, synthetic construct
CTPPSCCQLHHAGAGAGSGAGAGSGAGAGSGAGAGSGAGAGS

SEQ ID NO: 285 - protein, 40 aa, synthetic construct
SCCAPVYCCKGAGAGSGAGAGSGAGAGSGAGAGSGAGAGS

SEQ ID NO: 286 - protein, 19 aa, synthetic construct
  VARIANT 17: note = Any amino acid
  VARIANT 19: note = Any amino acid
GGVCGPSPPCITTGAGXGX

SEQ ID NO: 287 - protein, 16 aa, synthetic construct
  VARIANT 14: note = Any amino acid
  VARIANT 16: note = Any amino acid
GGVCGPSPPCGAGXGX

SEQ ID NO: 288 - protein, 16 aa, synthetic construct
  VARIANT 14: note = Any amino acid
  VARIANT 16: note = Any amino acid
CGPSPPCITTGAGXGX

SEQ ID NO: 289 - protein, 14 aa, synthetic construct
  VARIANT 12: note = Any amino acid
  VARIANT 14: note = Any amino acid
YGGSSGGGGAGXGX

SEQ ID NO: 290 - protein, 11 aa, synthetic construct
  VARIANT 9: note = Any amino acid
  VARIANT 11: note = Any amino acid
FGGGSGAGXGX

SEQ ID NO: 291 - protein, 17 aa, synthetic construct
  VARIANT 15: note = Any amino acid
  VARIANT 17: note = Any amino acid
CCQSSCCKPSCGAGXGX

SEQ ID NO: 292 - protein, 17 aa, synthetic construct
  VARIANT 15: note = Any amino acid
  VARIANT 17: note = Any amino acid
CVSSCCKPQCCGAGXGX

SEQ ID NO: 293 - protein, 16 aa, synthetic construct
  VARIANT 14: note = Any amino acid
  VARIANT 16: note = Any amino acid
PITCRRTCYHGAGXGX

SEQ ID NO: 294 - protein, 16 aa, synthetic construct
  VARIANT 14: note = Any amino acid
  VARIANT 16: note = Any amino acid
DCKLPCNPCAGAGXGX

SEQ ID NO: 295 - protein, 16 aa, synthetic construct
  VARIANT 14: note = Any amino acid
  VARIANT 16: note = Any amino acid
CLPCLPAASCGAGXGX

SEQ ID NO: 296 - protein, 16 aa, synthetic construct
  VARIANT 14: note = Any amino acid
  VARIANT 16: note = Any amino acid
CEPAICEPSCGAGXGX

SEQ ID NO: 297 - protein, 17 aa, synthetic construct
  VARIANT 15: note = Any amino acid
  VARIANT 17: note = Any amino acid
CQCSCCKPYCSGAGXGX

SEQ ID NO: 298 - protein, 17 aa, synthetic construct
  VARIANT 15: note = Any amino acid
  VARIANT 17: note = Any amino acid
FCGFPSCSTSCGAGXGX

SEQ ID NO: 299 - protein, 18 aa, synthetic construct
  VARIANT 16: note = Any amino acid
  VARIANT 18: note = Any amino acid
CTPPSCCQLHHAGAGXGX

SEQ ID NO: 300 - protein, 16 aa, synthetic construct
  VARIANT 14: note = Any amino acid
  VARIANT 16: note = Any amino acid
SCCAPVYCCKGAGXGX

SEQ ID NO: 301 - protein, 21 aa, synthetic construct
  VARIANT 14..21: note = This region may encompass one of the following sequences: GAGAGS or GAGSGA or GAGAGY or GAGYGA or GAGAGA or GAGAGV or GAGVGA or GAGAGVGY
GGVCGPSPPCITTXXXXXXXX

SEQ ID NO: 302 - protein, 18 aa, synthetic construct
  VARIANT 11..18: note = This region may encompass one of the following sequences: GAGAGS or GAGSGA or GAGAGY or GAGYGA or GAGAGA or GAGAGV or GAGVGA or GAGAGVGY
GGVCGPSPPCXXXXXXXX

SEQ ID NO: 303 - protein, 18 aa, synthetic construct
  VARIANT 11..18: note = This region may encompass one of the following sequences: GAGAGS or GAGSGA or GAGAGY or GAGYGA or GAGAGA or GAGAGV or GAGVGA or GAGAGVGY
CGPSPPCITTXXXXXXXX

SEQ ID NO: 304 - protein, 16 aa, synthetic construct
  VARIANT 9..16: note = This region may encompass one of the following sequences: GAGAGS or GAGSGA or GAGAGY or GAGYGA or GAGAGA or GAGAGV or GAGVGA or GAGAGVGY
YGGSSGGGXXXXXXXX

SEQ ID NO: 305 - protein, 13 aa, synthetic construct
  VARIANT 6..13: note = This region may encompass one of the following sequences: GAGAGS or GAGSGA or GAGAGY or GAGYGA or GAGAGA or GAGAGV or GAGVGA or GAGAGVGY
FGGGSXXXXXXXX

SEQ ID NO: 306 - protein, 19 aa, synthetic construct
  VARIANT 12..19: note = This region may encompass one of the following sequences: GAGAGS or GAGSGA or GAGAGY or GAGYGA or GAGAGA or GAGAGV or GAGVGA or GAGAGVGY
CCQSSCCKPSCXXXXXXXX

SEQ ID NO: 307 - protein, 19 aa, synthetic construct
  VARIANT 12..19: note = This region may encompass one of the following sequences: GAGAGS or GAGSGA or GAGAGY or GAGYGA or GAGAGA or GAGAGV or GAGVGA or GAGAGVGY
CVSSCCKPQCCXXXXXXXX

SEQ ID NO: 308 - protein, 18 aa, synthetic construct
  VARIANT 11..18: note = This region may encompass one of the following sequences: GAGAGS or GAGSGA or GAGAGY or GAGYGA or GAGAGA or GAGAGV or GAGVGA or GAGAGVGY
PITCRRTCYHXXXXXXXX

SEQ ID NO: 309 - protein, 18 aa, synthetic construct
  VARIANT 11..18: note = This region may encompass one of the following sequences: GAGAGS or GAGSGA or GAGAGY or GAGYGA or GAGAGA or GAGAGV or GAGVGA or GAGAGVGY
DCKLPCNPCAXXXXXXXX

SEQ ID NO: 310 - protein, 18 aa, synthetic construct
  VARIANT 11..18: note = This region may encompass one of the following sequences: GAGAGS or GAGSGA or GAGAGY or GAGYGA or GAGAGA or GAGAGV or GAGVGA or GAGAGVGY
CLPCLPAASCXXXXXXXX

SEQ ID NO: 311 - protein, 18 aa, synthetic construct
  VARIANT 11..18: note = This region may encompass one of the following sequences: GAGAGS or GAGSGA or GAGAGY or GAGYGA or GAGAGA or GAGAGV or GAGVGA or GAGAGVGY
CEPAICEPSCXXXXXXXX

SEQ ID NO: 312 - protein, 19 aa, synthetic construct
  VARIANT 12..19: note = This region may encompass one of the following sequences: GAGAGS or GAGSGA or GAGAGY or GAGYGA or GAGAGA or GAGAGV or GAGVGA or GAGAGVGY
CQCSCCKPYCSXXXXXXXX

SEQ ID NO: 313 - protein, 19 aa, synthetic construct
  VARIANT 12..19: note = This region may encompass one of the following sequences: GAGAGS or GAGSGA or GAGAGY or GAGYGA or GAGAGA or GAGAGV or GAGVGA or GAGAGVGY
FCGFPSCSTSCXXXXXXXX

SEQ ID NO: 314 - protein, 20 aa, synthetic construct
  VARIANT 13..20: note = This region may encompass one of the following sequences: GAGAGS or GAGSGA or GAGAGY or GAGYGA or GAGAGA or GAGAGV or GAGVGA or GAGAGVGY
CTPPSCCQLHHAXXXXXXXX

SEQ ID NO: 315 - protein, 18 aa, synthetic construct
  VARIANT 11..18: note = This region may encompass one of the following sequences: GAGAGS or GAGSGA or GAGAGY or GAGYGA or GAGAGA or GAGAGV or GAGVGA or GAGAGVGY
SCCAPVYCCKXXXXXXXX

SEQ ID NO: 316 - protein, 40 aa, synthetic construct
GGVCGPSPPCGPTGPTGPAGPRGLQGLQGLQGERGEQGPT

SEQ ID NO: 317 - protein, 40 aa, synthetic construct
CGPSPPCITTGPTGPTGPAGPRGLQGLQGLQGERGEQGPT

SEQ ID NO: 318 - protein, 38 aa, synthetic construct
YGGSSGGGGPTGPTGPAGPRGLQGLQGLQGERGEQGPT

SEQ ID NO: 319 - protein, 35 aa, synthetic construct
FGGGSGPTGPTGPAGPRGLQGLQGLQGERGEQGPT

SEQ ID NO: 320 - protein, 41 aa, synthetic construct
CCQSSCCKPSCGPTGPTGPAGPRGLQGLQGLQGERGEQGPT

SEQ ID NO: 321 - protein, 41 aa, synthetic construct
CVSSCCKPQCCGPTGPTGPAGPRGLQGLQGLQGERGEQGPT

SEQ ID NO: 322 - protein, 40 aa, synthetic construct
PITCRRTCYHGPTGPTGPAGPRGLQGLQGLQGERGEQGPT

SEQ ID NO: 323 - protein, 40 aa, synthetic construct
DCKLPCNPCAGPTGPTGPAGPRGLQGLQGLQGERGEQGPT

SEQ ID NO: 324 - protein, 40 aa, synthetic construct
CLPCLPAASCGPTGPTGPAGPRGLQGLQGLQGERGEQGPT

SEQ ID NO: 325 - protein, 40 aa, synthetic construct
CEPAICEPSCGPTGPTGPAGPRGLQGLQGLQGERGEQGPT

SEQ ID NO: 326 - protein, 41 aa, synthetic construct
CQCSCCKPYCSGPTGPTGPAGPRGLQGLQGLQGERGEQGPT

SEQ ID NO: 327 - protein, 41 aa, synthetic construct
FCGFPSCSTSCGPTGPTGPAGPRGLQGLQGLQGERGEQGPT

SEQ ID NO: 328 - protein, 42 aa, synthetic construct
CTPPSCCQLHHAGPTGPTGPAGPRGLQGLQGLQGERGEQGPT

SEQ ID NO: 329 - protein, 40 aa, synthetic construct
SCCAPVYCCKGPTGPTGPAGPRGLQGLQGLQGERGEQGPT

SEQ ID NO: 330 - protein, 19 aa, synthetic construct
GGVCGPSPPCITTGPTGPT

SEQ ID NO: 331 - protein, 16 aa, synthetic construct
GGVCGPSPPCGPTGPT

SEQ ID NO: 332 - protein, 16 aa, synthetic construct
CGPSPPCITTGPTGPT

SEQ ID NO: 333 - protein, 14 aa, synthetic construct
YGGSSGGGGPTGPT

SEQ ID NO: 334 - protein, 11 aa, synthetic construct
FGGGSGPTGPT

SEQ ID NO: 335 - protein, 17 aa, synthetic construct
CCQSSCCKPSCGPTGPT

SEQ ID NO: 336 - protein, 17 aa, synthetic construct
CVSSCCKPQCCGPTGPT

SEQ ID NO: 337 - protein, 16 aa, synthetic construct
PITCRRTCYHGPTGPT

SEQ ID NO: 338 - protein, 16 aa, synthetic construct
DCKLPCNPCAGPTGPT

SEQ ID NO: 339 - protein, 16 aa, synthetic construct
CLPCLPAASCGPTGPT

SEQ ID NO: 340 - protein, 16 aa, synthetic construct
CEPAICEPSCGPTGPT

SEQ ID NO: 341 - protein, 17 aa, synthetic construct
CQCSCCKPYCSGPTGPT

SEQ ID NO: 342 - protein, 17 aa, synthetic construct
FCGFPSCSTSCGPTGPT

SEQ ID NO: 343 - protein, 18 aa, synthetic construct
CTPPSCCQLHHAGPTGPT

SEQ ID NO: 344 - protein, 16 aa, synthetic construct
SCCAPVYCCKGPTGPT

SEQ ID NO: 345 - protein, 19 aa, synthetic construct
GGVCGPSPPCITTGLQGLQ

SEQ ID NO: 346 - protein, 16 aa, synthetic construct
GGVCGPSPPCGLQGLQ

SEQ ID NO: 347 - protein, 16 aa, synthetic construct
CGPSPPCITTGLQGLQ

SEQ ID NO: 348 - protein, 14 aa, synthetic construct
YGGSSGGGGLQGLQ

SEQ ID NO: 349 - protein, 11 aa, synthetic construct
FGGGSGLQGLQ

SEQ ID NO: 350 - protein, 17 aa, synthetic construct
CCQSSCCKPSCGLQGLQ

SEQ ID NO: 351 - protein, 17 aa, synthetic construct
CVSSCCKPQCCGLQGLQ

SEQ ID NO: 352 - protein, 16 aa, synthetic construct
PITCRRTCYHGLQGLQ

SEQ ID NO: 353 - protein, 16 aa, synthetic construct
DCKLPCNPCAGLQGLQ

SEQ ID NO: 354 - protein, 16 aa, synthetic construct
CLPCLPAASCGLQGLQ

SEQ ID NO: 355 - protein, 16 aa, synthetic construct
CEPAICEPSCGLQGLQ

SEQ ID NO: 356 - protein, 17 aa, synthetic construct
CQCSCCKPYCSGLQGLQ

SEQ ID NO: 357 - protein, 17 aa, synthetic construct
FCGFPSCSTSCGLQGLQ

SEQ ID NO: 358 - protein, 18 aa, synthetic construct
CTPPSCCQLHHAGLQGLQ

SEQ ID NO: 359 - protein, 16 aa, synthetic construct
SCCAPVYCCKGLQGLQ

SEQ ID NO: 360 - protein, 19 aa, synthetic construct
  VARIANT 14..19: note = This region may encompass one of the following sequences: GXPGXP, wherein each X is independently any amino acid or GXPGXP, wherein each X is 4-hydroxyproline or GPAGPA
GGVCGPSPPCITTXXXXXX

SEQ ID NO: 361 - protein, 16 aa, synthetic construct
  VARIANT 11..16: note = This region may encompass one of the following sequences: GXPGXP, wherein each X is independently any amino acid or GXPGXP, wherein each X is 4-hydroxyproline or GPAGPA
GGVCGPSPPCXXXXXX

SEQ ID NO: 362 - protein, 16 aa, synthetic construct
  VARIANT 11..16: note = This region may encompass one of the following sequences: GXPGXP, wherein each X is independently any amino acid or GXPGXP, wherein each X is 4-hydroxyproline or GPAGPA
CGPSPPCITTXXXXXX

SEQ ID NO: 363 - protein, 14 aa, synthetic construct
  VARIANT 9..14: note = This region may encompass one of the following sequences: GXPGXP, wherein each X is independently any amino acid or GXPGXP, wherein each X is 4-hydroxyproline or GPAGPA
YGGSSGGGXXXXXX

SEQ ID NO: 364 - protein, 11 aa, synthetic construct
  VARIANT 6..11: note = This region may encompass one of the following sequences: GXPGXP, wherein each X is independently any amino acid or GXPGXP, wherein each X is 4-hydroxyproline or GPAGPA
FGGGSXXXXXX

SEQ ID NO: 365 - protein, 17 aa, synthetic construct
  VARIANT 12..17: note = This region may encompass one of the following sequences: GXPGXP, wherein each X is independently any amino acid or GXPGXP, wherein each X is 4-hydroxyproline or GPAGPA
CCQSSCCKPSCXXXXXX

SEQ ID NO: 366 - protein, 17 aa, synthetic construct
  VARIANT 12..17: note = This region may encompass one of the following sequences: GXPGXP, wherein each X is independently any amino acid or GXPGXP, wherein each X is 4-hydroxyproline or GPAGPA
CVSSCCKPQCCXXXXXX

SEQ ID NO: 367 - protein, 16 aa, synthetic construct
  VARIANT 11..16: note = This region may encompass one of the following sequences: GXPGXP, wherein each X is independently any amino acid or GXPGXP, wherein each X is 4-hydroxyproline or GPAGPA
PITCRRTCYHXXXXXX

SEQ ID NO: 368 - protein, 16 aa, synthetic construct
  VARIANT 11..16: note = This region may encompass one of the following sequences: GXPGXP, wherein each X is independently any amino acid or GXPGXP, wherein each X is 4-hydroxyproline or GPAGPA
DCKLPCNPCAXXXXXX

SEQ ID NO: 369 - protein, 16 aa, synthetic construct
  VARIANT 11..16: note = This region may encompass one of the following sequences: GXPGXP, wherein each X is independently any amino acid or GXPGXP, wherein each X is 4-hydroxyproline or GPAGPA
CLPCLPAASCXXXXXX

SEQ ID NO: 370 - protein, 16 aa, synthetic construct
  VARIANT 11..16: note = This region may encompass one of the following sequences: GXPGXP, wherein each X is independently any amino acid or GXPGXP, wherein each X is 4-hydroxyproline or GPAGPA
CEPAICEPSCXXXXXX

SEQ ID NO: 371 - protein, 17 aa, synthetic construct
  VARIANT 12..17: note = This region may encompass one of the following sequences: GXPGXP, wherein each X is independently any amino acid or GXPGXP, wherein each X is 4-hydroxyproline or GPAGPA
CQCSCCKPYCSXXXXXX

SEQ ID NO: 372 - protein, 17 aa, synthetic construct
  VARIANT 12..17: note = This region may encompass one of the following sequences: GXPGXP, wherein each X is independently any amino acid or GXPGXP, wherein each X is 4-hydroxyproline or GPAGPA
FCGFPSCSTSCXXXXXX

SEQ ID NO: 373 - protein, 18 aa, synthetic construct
  VARIANT 13..18: note = This region may encompass one of the following sequences: GXPGXP, wherein each X is independently any amino acid or GXPGXP, wherein each X is 4-hydroxyproline or GPAGPA
CTPPSCCQLHHAXXXXXX

SEQ ID NO: 374 - protein, 16 aa, synthetic construct
  VARIANT 11..16: note = This region may encompass one of the following sequences: GXPGXP, wherein each X is independently any amino acid or GXPGXP, wherein each X is 4-hydroxyproline or GPAGPA
SCCAPVYCCKXXXXXX

SEQ ID NO: 375 - protein, 25 aa, synthetic construct
GGVCGPSPPCGGRPSDSYGAPGGGN

SEQ ID NO: 376 - protein, 25 aa, synthetic construct
CGPSPPCITTGGRPSDSYGAPGGGN

SEQ ID NO: 377 - protein, 23 aa, synthetic construct
YGGSSGGGGGRPSDSYGAPGGGN

SEQ ID NO: 378 - protein, 20 aa, synthetic construct
FGGGSGGRPSDSYGAPGGGN

SEQ ID NO: 379 - protein, 26 aa, synthetic construct
CCQSSCCKPSCGGRPSDSYGAPGGGN

SEQ ID NO: 380 - protein, 26 aa, synthetic construct
CVSSCCKPQCCGGRPSDSYGAPGGGN

SEQ ID NO: 381 - protein, 25 aa, synthetic construct
PITCRRTCYHGGRPSDSYGAPGGGN

SEQ ID NO: 382 - protein, 25 aa, synthetic construct
DCKLPCNPCAGGRPSDSYGAPGGGN

SEQ ID NO: 383 - protein, 25 aa, synthetic construct
CLPCLPAASCGGRPSDSYGAPGGGN

SEQ ID NO: 384 - protein, 25 aa, synthetic construct
CEPAICEPSCGGRPSDSYGAPGGGN

SEQ ID NO: 385 - protein, 26 aa, synthetic construct
CQCSCCKPYCSGGRPSDSYGAPGGGN

SEQ ID NO: 386 - protein, 26 aa, synthetic construct
FCGFPSCSTSCGGRPSDSYGAPGGGN

SEQ ID NO: 387 - protein, 27 aa, synthetic construct
CTPPSCCQLHHAGGRPSDSYGAPGGGN

SEQ ID NO: 388 - protein, 25 aa, synthetic construct
SCCAPVYCCKGGRPSDSYGAPGGGN

SEQ ID NO: 389 - protein, 24 aa, synthetic construct
GGVCGPSPPCITTGAPAQTPSSQY

SEQ ID NO: 390 - protein, 21 aa, synthetic construct
GGVCGPSPPCGAPAQTPSSQY

SEQ ID NO: 391 - protein, 21 aa, synthetic construct
CGPSPPCITTGAPAQTPSSQY

SEQ ID NO: 392 - protein, 19 aa, synthetic construct
YGGSSGGGGAPAQTPSSQY

SEQ ID NO: 393 - protein, 16 aa, synthetic construct
FGGGSGAPAQTPSSQY

SEQ ID NO: 394 - protein, 22 aa, synthetic construct
CCQSSCCKPSCGAPAQTPSSQY

SEQ ID NO: 395 - protein, 22 aa, synthetic construct
CVSSCCKPQCCGAPAQTPSSQY

SEQ ID NO: 396 - protein, 21 aa, synthetic construct
PITCRRTCYHGAPAQTPSSQY

SEQ ID NO: 397 - protein, 21 aa, synthetic construct
DCKLPCNPCAGAPAQTPSSQY

SEQ ID NO: 398 - protein, 21 aa, synthetic construct
CLPCLPAASCGAPAQTPSSQY

SEQ ID NO: 399 - protein, 21 aa, synthetic construct
CEPAICEPSCGAPAQTPSSQY

SEQ ID NO: 400 - protein, 22 aa, synthetic construct
CQCSCCKPYCSGAPAQTPSSQY

SEQ ID NO: 401 - protein, 22 aa, synthetic construct
FCGFPSCSTSCGAPAQTPSSQY

SEQ ID NO: 402 - protein, 23 aa, synthetic construct
CTPPSCCQLHHAGAPAQTPSSQY

SEQ ID NO: 403 - protein, 21 aa, synthetic construct
SCCAPVYCCKGAPAQTPSSQY

SEQ ID NO: 404 - protein, 24 aa, synthetic construct
GGVCGPSPPCITTAQTPSSQYGAP

SEQ ID NO: 405 - protein, 21 aa, synthetic construct
GGVCGPSPPCAQTPSSQYGAP

SEQ ID NO: 406 - protein, 21 aa, synthetic construct
CGPSPPCITTAQTPSSQYGAP

SEQ ID NO: 407 - protein, 19 aa, synthetic construct
YGGSSGGGAQTPSSQYGAP

SEQ ID NO: 408 - protein, 16 aa, synthetic construct
FGGGSAQTPSSQYGAP

SEQ ID NO: 409 - protein, 22 aa, synthetic construct
CCQSSCCKPSCAQTPSSQYGAP

SEQ ID NO: 410 - protein, 22 aa, synthetic construct
CVSSCCKPQCCAQTPSSQYGAP

SEQ ID NO: 411 - protein, 21 aa, synthetic construct
PITCRRTCYHAQTPSSQYGAP

SEQ ID NO: 412 - protein, 21 aa, synthetic construct
DCKLPCNPCAAQTPSSQYGAP

SEQ ID NO: 413 - protein, 21 aa, synthetic construct
CLPCLPAASCAQTPSSQYGAP

SEQ ID NO: 414 - protein, 21 aa, synthetic construct
CEPAICEPSCAQTPSSQYGAP

SEQ ID NO: 415 - protein, 22 aa, synthetic construct
CQCSCCKPYCSAQTPSSQYGAP

SEQ ID NO: 416 - protein, 22 aa, synthetic construct
FCGFPSCSTSCAQTPSSQYGAP

SEQ ID NO: 417 - protein, 23 aa, synthetic construct
CTPPSCCQLHHAAQTPSSQYGAP

SEQ ID NO: 418 - protein, 21 aa, synthetic construct
SCCAPVYCCKAQTPSSQYGAP

SEQ ID NO: 419 - protein, 40 aa, synthetic construct
GGVCGPSPPCGGFGGMGGGSGGFGGMGGGSGGFGGMGGGS

SEQ ID NO: 420 - protein, 40 aa, synthetic construct
CGPSPPCITTGGFGGMGGGSGGFGGMGGGSGGFGGMGGGS

SEQ ID NO: 421 - protein, 38 aa, synthetic construct
YGGSSGGGGGFGGMGGGSGGFGGMGGGSGGFGGMGGGS

SEQ ID NO: 422 - protein, 35 aa, synthetic construct
FGGGSGGFGGMGGGSGGFGGMGGGSGGFGGMGGGS

SEQ ID NO: 423 - protein, 41 aa, synthetic construct
CCQSSCCKPSCGGFGGMGGGSGGFGGMGGGSGGFGGMGGGS

SEQ ID NO: 424 - protein, 41 aa, synthetic construct
CVSSCCKPQCCGGFGGMGGGSGGFGGMGGGSGGFGGMGGGS

SEQ ID NO: 425 - protein, 40 aa, synthetic construct
PITCRRTCYHGGFGGMGGGSGGFGGMGGGSGGFGGMGGGS

SEQ ID NO: 426 - protein, 40 aa, synthetic construct
DCKLPCNPCAGGFGGMGGGSGGFGGMGGGSGGFGGMGGGS

SEQ ID NO: 427 - protein, 40 aa, synthetic construct
CLPCLPAASCGGFGGMGGGSGGFGGMGGGSGGFGGMGGGS

SEQ ID NO: 428 - protein, 40 aa, synthetic construct
CEPAICEPSCGGFGGMGGGSGGFGGMGGGSGGFGGMGGGS

SEQ ID NO: 429 - protein, 41 aa, synthetic construct
CQCSCCKPYCSGGFGGMGGGSGGFGGMGGGSGGFGGMGGGS

SEQ ID NO: 430 - protein, 41 aa, synthetic construct
FCGFPSCSTSCGGFGGMGGGSGGFGGMGGGSGGFGGMGGGS

SEQ ID NO: 431 - protein, 42 aa, synthetic construct
CTPPSCCQLHHAGGFGGMGGGSGGFGGMGGGSGGFGGMGGGS

SEQ ID NO: 432 - protein, 40 aa, synthetic construct
SCCAPVYCCKGGFGGMGGGSGGFGGMGGGSGGFGGMGGGS

SEQ ID NO: 433 - protein, 17 aa, synthetic construct
GGVCGPSPPCITTMGGG

SEQ ID NO: 434 - protein, 14 aa, synthetic construct
GGVCGPSPPCMGGG

SEQ ID NO: 435 - protein, 14 aa, synthetic construct
CGPSPPCITTMGGG

SEQ ID NO: 436 - protein, 12 aa, synthetic construct
YGGSSGGGMGGG

SEQ ID NO: 437 - protein, 9 aa, synthetic construct
FGGGSMGGG

SEQ ID NO: 438 - protein, 15 aa, synthetic construct
CCQSSCCKPSCMGGG

SEQ ID NO: 439 - protein, 15 aa, synthetic construct
CVSSCCKPQCCMGGG

SEQ ID NO: 440 - protein, 14 aa, synthetic construct
PITCRRTCYHMGGG

SEQ ID NO: 441 - protein, 14 aa, synthetic construct
DCKLPCNPCAMGGG

SEQ ID NO: 442 - protein, 14 aa, synthetic construct
CLPCLPAASCMGGG

SEQ ID NO: 443 - protein, 14 aa, synthetic construct
CEPAICEPSCMGGG

SEQ ID NO: 444 - protein, 15 aa, synthetic construct
CQCSCCKPYCSMGGG

SEQ ID NO: 445 - protein, 15 aa, synthetic construct
FCGFPSCSTSCMGGG

SEQ ID NO: 446 - protein, 16 aa, synthetic construct
CTPPSCCQLHHAMGGG

SEQ ID NO: 447 - protein, 14 aa, synthetic construct
SCCAPVYCCKMGGG

SEQ ID NO: 448 - protein, 18 aa, synthetic construct
GGVCGPSPPCITTFGGMG

SEQ ID NO: 449 - protein, 15 aa, synthetic construct
GGVCGPSPPCFGGMG

SEQ ID NO: 450 - protein, 15 aa, synthetic construct
CGPSPPCITTFGGMG

SEQ ID NO: 451 - protein, 13 aa, synthetic construct
YGGSSGGGFGGMG

SEQ ID NO: 452 - protein, 10 aa, synthetic construct
FGGGSFGGMG

SEQ ID NO: 453 - protein, 16 aa, synthetic construct
CCQSSCCKPSCFGGMG

SEQ ID NO: 454 - protein, 16 aa, synthetic construct
CVSSCCKPQCCFGGMG

SEQ ID NO: 455 - protein, 15 aa, synthetic construct
PITCRRTCYHFGGMG

SEQ ID NO: 456 - protein, 15 aa, synthetic construct
DCKLPCNPCAFGGMG

SEQ ID NO: 457 - protein, 15 aa, synthetic construct
CLPCLPAASCFGGMG

SEQ ID NO: 458 - protein, 15 aa, synthetic construct
CEPAICEPSCFGGMG

SEQ ID NO: 459 - protein, 16 aa, synthetic construct
CQCSCCKPYCSFGGMG

SEQ ID NO: 460 - protein, 16 aa, synthetic construct
FCGFPSCSTSCFGGMG

SEQ ID NO: 461 - protein, 17 aa, synthetic construct
CTPPSCCQLHHAFGGMG

SEQ ID NO: 462 - protein, 15 aa, synthetic construct
SCCAPVYCCKFGGMG

SEQ ID NO: 463 - protein, 23 aa, synthetic construct
  VARIANT 14..23: note = This region may encompass one of the following sequences: GGFGGMGGGS or FGGMGGG or GGFGGMGGG or FGGMGGGNAG
GGVCGPSPPCITTXXXXXXXXXX

SEQ ID NO: 464 - protein, 20 aa, synthetic construct
  VARIANT 11..20: note = This region may encompass one of the following sequences: GGFGGMGGGS or FGGMGGG or GGFGGMGGG or FGGMGGGNAG
GGVCGPSPPCXXXXXXXXXX

SEQ ID NO: 465 - protein, 20 aa, synthetic construct
  VARIANT 11..20: note = This region may encompass one of the following sequences: GGFGGMGGGS or FGGMGGG or GGFGGMGGG or FGGMGGGNAG
CGPSPPCITTXXXXXXXXXX

SEQ ID NO: 466 - protein, 18 aa, synthetic construct
  VARIANT 9..18: note = This region may encompass one of the following sequences: GGFGGMGGGS or FGGMGGG or GGFGGMGGG or FGGMGGGNAG
YGGSSGGGXXXXXXXXXX

SEQ ID NO: 467 - protein, 15 aa, synthetic construct
  VARIANT 6..15: note = This region may encompass one of the following sequences: GGFGGMGGGS or FGGMGGG or GGFGGMGGG or FGGMGGGNAG
FGGGSXXXXXXXXXX

SEQ ID NO: 468 - protein, 21 aa, synthetic construct
  VARIANT 12..21: note = This region may encompass one of the following sequences: GGFGGMGGGS or FGGMGGG or GGFGGMGGG or FGGMGGGNAG
CCQSSCCKPSCXXXXXXXXXX

SEQ ID NO: 469 - protein, 21 aa, synthetic construct
  VARIANT 12..21: note = This region may encompass one of the following sequences: GGFGGMGGGS or FGGMGGG or GGFGGMGGG or FGGMGGGNAG
CVSSCCKPQCCXXXXXXXXXX

SEQ ID NO: 470 - protein, 20 aa, synthetic construct
  VARIANT 11..20: note = This region may encompass one of the following sequences: GGFGGMGGGS or FGGMGGG or GGFGGMGGG or FGGMGGGNAG
PITCRRTCYHXXXXXXXXXX

SEQ ID NO: 471 - protein, 20 aa, synthetic construct
  VARIANT 11..20: note = This region may encompass one of the following sequences: GGFGGMGGGS or FGGMGGG or GGFGGMGGG or FGGMGGGNAG
DCKLPCNPCAXXXXXXXXXX

SEQ ID NO: 472 - protein, 20 aa, synthetic construct
  VARIANT 11..20: note = This region may encompass one of the following sequences: GGFGGMGGGS or FGGMGGG or GGFGGMGGG or FGGMGGGNAG
CLPCLPAASCXXXXXXXXXX

SEQ ID NO: 473 - protein, 20 aa, synthetic construct
  VARIANT 11..20: note = This region may encompass one of the following sequences: GGFGGMGGGS or FGGMGGG or GGFGGMGGG or FGGMGGGNAG
CEPAICEPSCXXXXXXXXXX

SEQ ID NO: 474 - protein, 21 aa, synthetic construct
  VARIANT 12..21: note = This region may encompass one of the following sequences: GGFGGMGGGS or FGGMGGG or GGFGGMGGG or FGGMGGGNAG
CQCSCCKPYCSXXXXXXXXXX

SEQ ID NO: 475 - protein, 21 aa, synthetic construct
  VARIANT 12..21: note = This region may encompass one of the following sequences: GGFGGMGGGS or FGGMGGG or GGFGGMGGG or FGGMGGGNAG
FCGFPSCSTSCXXXXXXXXXX

SEQ ID NO: 476 - protein, 22 aa, synthetic construct
  VARIANT 13..22: note = This region may encompass one of the following sequences: GGFGGMGGGS or FGGMGGG or GGFGGMGGG or FGGMGGGNAG
CTPPSCCQLHHAXXXXXXXXXX

SEQ ID NO: 477 - protein, 20 aa, synthetic construct
  VARIANT 11..20: note = This region may encompass one of the following sequences: GGFGGMGGGS or FGGMGGG or GGFGGMGGG or FGGMGGGNAG
SCCAPVYCCKXXXXXXXXXX

SEQ ID NO: 478 - protein, 40 aa, synthetic construct
GGVCGPSPPCGQGQGQGQGQGQGQGQGQGQGQGQGQGQGQ

SEQ ID NO: 479 - protein, 40 aa, synthetic construct
CGPSPPCITTGQGQGQGQGQGQGQGQGQGQGQGQGQGQGQ

SEQ ID NO: 480 - protein, 38 aa, synthetic construct
YGGSSGGGGQGQGQGQGQGQGQGQGQGQGQGQGQGQGQ

SEQ ID NO: 481 - protein, 35 aa, synthetic construct
FGGGSGQGQGQGQGQGQGQGQGQGQGQGQGQGQGQ

SEQ ID NO: 482 - protein, 41 aa, synthetic construct
CCQSSCCKPSCGQGQGQGQGQGQGQGQGQGQGQGQGQGQGQ

SEQ ID NO: 483 - protein, 41 aa, synthetic construct
CVSSCCKPQCCGQGQGQGQGQGQGQGQGQGQGQGQGQGQGQ

SEQ ID NO: 484 - protein, 40 aa, synthetic construct
PITCRRTCYHGQGQGQGQGQGQGQGQGQGQGQGQGQGQGQ

SEQ ID NO: 485 - protein, 40 aa, synthetic construct
DCKLPCNPCAGQGQGQGQGQGQGQGQGQGQGQGQGQGQGQ

SEQ ID NO: 486 - protein, 40 aa, synthetic construct
CLPCLPAASCGQGQGQGQGQGQGQGQGQGQGQGQGQGQGQ

SEQ ID NO: 487 - protein, 40 aa, synthetic construct
CEPAICEPSCGQGQGQGQGQGQGQGQGQGQGQGQGQGQGQ

SEQ ID NO: 488 - protein, 41 aa, synthetic construct
CQCSCCKPYCSGQGQGQGQGQGQGQGQGQGQGQGQGQGQGQ

SEQ ID NO: 489 - protein, 41 aa, synthetic construct
FCGFPSCSTSCGQGQGQGQGQGQGQGQGQGQGQGQGQGQGQ

SEQ ID NO: 490 - protein, 42 aa, synthetic construct
CTPPSCCQLHHAGQGQGQGQGQGQGQGQGQGQGQGQGQGQGQ

SEQ ID NO: 491 - protein, 40 aa, synthetic construct
SCCAPVYCCKGQGQGQGQGQGQGQGQGQGQGQGQGQGQGQ

SEQ ID NO: 492 - protein, 40 aa, synthetic construct
GGVCGPSPPCAKAKAKAKAKAKAKAKAKAKAKAKAKAKAK

SEQ ID NO: 493 - protein, 40 aa, synthetic construct
CGPSPPCITTAKAKAKAKAKAKAKAKAKAKAKAKAKAKAK

SEQ ID NO: 494 - protein, 38 aa, synthetic construct
YGGSSGGGAKAKAKAKAKAKAKAKAKAKAKAKAKAKAK

SEQ ID NO: 495 - protein, 35 aa, synthetic construct
FGGGSAKAKAKAKAKAKAKAKAKAKAKAKAKAKAK

SEQ ID NO: 496 - protein, 41 aa, synthetic construct
CCQSSCCKPSCAKAKAKAKAKAKAKAKAKAKAKAKAKAKAK

SEQ ID NO: 497 - protein, 41 aa, synthetic construct
CVSSCCKPQCCAKAKAKAKAKAKAKAKAKAKAKAKAKAKAK

SEQ ID NO: 498 - protein, 40 aa, synthetic construct
PITCRRTCYHAKAKAKAKAKAKAKAKAKAKAKAKAKAKAK

SEQ ID NO: 499 - protein, 40 aa, synthetic construct
DCKLPCNPCAAKAKAKAKAKAKAKAKAKAKAKAKAKAKAK

SEQ ID NO: 500 - protein, 40 aa, synthetic construct
CLPCLPAASCAKAKAKAKAKAKAKAKAKAKAKAKAKAKAK

SEQ ID NO: 501 - protein, 40 aa, synthetic construct
CEPAICEPSCAKAKAKAKAKAKAKAKAKAKAKAKAKAKAK

SEQ ID NO: 502 - protein, 41 aa, synthetic construct
CQCSCCKPYCSAKAKAKAKAKAKAKAKAKAKAKAKAKAKAK

SEQ ID NO: 503 - protein, 41 aa, synthetic construct
FCGFPSCSTSCAKAKAKAKAKAKAKAKAKAKAKAKAKAKAK

SEQ ID NO: 504 - protein, 42 aa, synthetic construct
CTPPSCCQLHHAAKAKAKAKAKAKAKAKAKAKAKAKAKAKAK

SEQ ID NO: 505 - protein, 40 aa, synthetic construct
SCCAPVYCCKAKAKAKAKAKAKAKAKAKAKAKAKAKAKAK

SEQ ID NO: 506 - protein, 40 aa, synthetic construct
GGVCGPSPPCLKLKLKLKLKLKLKLKLKLKLKLKLKLKLK

SEQ ID NO: 507 - protein, 40 aa, synthetic construct
CGPSPPCITTLKLKLKLKLKLKLKLKLKLKLKLKLKLKLK

SEQ ID NO: 508 - protein, 38 aa, synthetic construct
YGGSSGGGLKLKLKLKLKLKLKLKLKLKLKLKLKLKLK

SEQ ID NO: 509 - protein, 35 aa, synthetic construct
FGGGSLKLKLKLKLKLKLKLKLKLKLKLKLKLKLK

SEQ ID NO: 510 - protein, 41 aa, synthetic construct
CCQSSCCKPSCLKLKLKLKLKLKLKLKLKLKLKLKLKLKLK

SEQ ID NO: 511 - protein, 41 aa, synthetic construct
CVSSCCKPQCCLKLKLKLKLKLKLKLKLKLKLKLKLKLKLK

SEQ ID NO: 512 - protein, 40 aa, synthetic construct
PITCRRTCYHLKLKLKLKLKLKLKLKLKLKLKLKLKLKLK

SEQ ID NO: 513 - protein, 40 aa, synthetic construct
DCKLPCNPCALKLKLKLKLKLKLKLKLKLKLKLKLKLKLK

SEQ ID NO: 514 - protein, 40 aa, synthetic construct
CLPCLPAASCLKLKLKLKLKLKLKLKLKLKLKLKLKLKLK

SEQ ID NO: 515 - protein, 40 aa, synthetic construct
CEPAICEPSCLKLKLKLKLKLKLKLKLKLKLKLKLKLKLK

SEQ ID NO: 516 - protein, 41 aa, synthetic construct
CQCSCCKPYCSLKLKLKLKLKLKLKLKLKLKLKLKLKLKLK

SEQ ID NO: 517 - protein, 41 aa, synthetic construct
FCGFPSCSTSCLKLKLKLKLKLKLKLKLKLKLKLKLKLKLK

SEQ ID NO: 518 - protein, 42 aa, synthetic construct
CTPPSCCQLHHALKLKLKLKLKLKLKLKLKLKLKLKLKLKLK

SEQ ID NO: 519 - protein, 40 aa, synthetic construct
SCCAPVYCCKLKLKLKLKLKLKLKLKLKLKLKLKLKLKLK

SEQ ID NO: 520 - protein, 40 aa, synthetic construct
GGVCGPSPPCGAGAGAGAGAGAGAGAGAGAGAGAGAGAGA

SEQ ID NO: 521 - protein, 40 aa, synthetic construct
CGPSPPCITTGAGAGAGAGAGAGAGAGAGAGAGAGAGAGA

SEQ ID NO: 522 - protein, 38 aa, synthetic construct
YGGSSGGGGAGAGAGAGAGAGAGAGAGAGAGAGAGAGA

SEQ ID NO: 523 - protein, 35 aa, synthetic construct
FGGGSGAGAGAGAGAGAGAGAGAGAGAGAGAGAGA

SEQ ID NO: 524 - protein, 41 aa, synthetic construct
CCQSSCCKPSCGAGAGAGAGAGAGAGAGAGAGAGAGAGAGA

SEQ ID NO: 525 - protein, 41 aa, synthetic construct
CVSSCCKPQCCGAGAGAGAGAGAGAGAGAGAGAGAGAGAGA

SEQ ID NO: 526 - protein, 40 aa, synthetic construct
PITCRRTCYHGAGAGAGAGAGAGAGAGAGAGAGAGAGAGA

SEQ ID NO: 527 - protein, 40 aa, synthetic construct
DCKLPCNPCAGAGAGAGAGAGAGAGAGAGAGAGAGAGAGA

SEQ ID NO: 528 - protein, 40 aa, synthetic construct
CLPCLPAASCGAGAGAGAGAGAGAGAGAGAGAGAGAGAGA

SEQ ID NO: 529 - protein, 40 aa, synthetic construct
CEPAICEPSCGAGAGAGAGAGAGAGAGAGAGAGAGAGAGA

SEQ ID NO: 530 - protein, 41 aa, synthetic construct
CQCSCCKPYCSGAGAGAGAGAGAGAGAGAGAGAGAGAGAGA

SEQ ID NO: 531 - protein, 41 aa, synthetic construct
FCGFPSCSTSCGAGAGAGAGAGAGAGAGAGAGAGAGAGAGA

SEQ ID NO: 532 - protein, 42 aa, synthetic construct
CTPPSCCQLHHAGAGAGAGAGAGAGAGAGAGAGAGAGAGAGA

SEQ ID NO: 533 - protein, 40 aa, synthetic construct
SCCAPVYCCKGAGAGAGAGAGAGAGAGAGAGAGAGAGAGA

SEQ ID NO: 534 - protein, 53 aa, synthetic construct
  VARIANT 14..53: note = This region may encompass one of the following sequences: (GQ)n, where n is 1-20 or (AK)n, where n is 1-20 or (LK)n, where n is 1-20 or (GA)n, where n is 1-20
GGVCGPSPPCITTXXXXXXXXXXXXXXXXXXXXXXXXXXXXXXXXXXXXXXXX

SEQ ID NO: 535 - protein, 50 aa, synthetic construct
  VARIANT 11..50: note = This region may encompass one of the following sequences: (GQ)n, where n is 1-20 or (AK)n, where n is 1-20 or (LK)n, where n is 1-20 or (GA)n, where n is 1-20
GGVCGPSPPCXXXXXXXXXXXXXXXXXXXXXXXXXXXXXXXXXXXXXXXX

SEQ ID NO: 536 - protein, 50 aa, synthetic construct
  VARIANT 11..50: note = This region may encompass one of the following sequences: (GQ)n, where n is 1-20 or (AK)n, where n is 1-20 or (LK)n, where n is 1-20 or (GA)n, where n is 1-20
CGPSPPCITTXXXXXXXXXXXXXXXXXXXXXXXXXXXXXXXXXXXXXXXX

SEQ ID NO: 537 - protein, 48 aa, synthetic construct
  VARIANT 9..48: note = This region may encompass one of the following sequences: (GQ)n, where n is 1-20 or (AK)n, where n is 1-20 or (LK)n, where n is 1-20 or (GA)n, where n is 1-20
YGGSSGGGXXXXXXXXXXXXXXXXXXXXXXXXXXXXXXXXXXXXXXXX

SEQ ID NO: 538 - protein, 45 aa, synthetic construct
  VARIANT 6..45: note = This region may encompass one of the following sequences: (GQ)n, where n is 1-20 or (AK)n, where n is 1-20 or (LK)n, where n is 1-20 or (GA)n, where n is 1-20
FGGGSXXXXXXXXXXXXXXXXXXXXXXXXXXXXXXXXXXXXXXXX

SEQ ID NO: 539 - protein, 51 aa, synthetic construct
  VARIANT 12..51: note = This region may encompass one of the following sequences: (GQ)n, where n is 1-20 or (AK)n, where n is 1-20 or (LK)n, where n is 1-20 or (GA)n, where n is 1-20
CCQSSCCKPSCXXXXXXXXXXXXXXXXXXXXXXXXXXXXXXXXXXXXXXXX

SEQ ID NO: 540 - protein, 51 aa, synthetic construct
  VARIANT 12..51: note = This region may encompass one of the following sequences: (GQ)n, where n is 1-20 or (AK)n, where n is 1-20 or (LK)n, where n is 1-20 or (GA)n, where n is 1-20
CVSSCCKPQCCXXXXXXXXXXXXXXXXXXXXXXXXXXXXXXXXXXXXXXXX

SEQ ID NO: 541 - protein, 50 aa, synthetic construct
  VARIANT 11..50: note = This region may encompass one of the following sequences: (GQ)n, where n is 1-20 or (AK)n, where n is 1-20 or (LK)n, where n is 1-20 or (GA)n, where n is 1-20
PITCRRTCYHXXXXXXXXXXXXXXXXXXXXXXXXXXXXXXXXXXXXXXXX

SEQ ID NO: 542 - protein, 50 aa, synthetic construct
  VARIANT 11..50: note = This region may encompass one of the following sequences: (GQ)n, where n is 1-20 or (AK)n, where n is 1-20 or (LK)n, where n is 1-20 or (GA)n, where n is 1-20
DCKLPCNPCAXXXXXXXXXXXXXXXXXXXXXXXXXXXXXXXXXXXXXXXX

SEQ ID NO: 543 - protein, 50 aa, synthetic construct
  VARIANT 11..50: note = This region may encompass one of the following sequences: (GQ)n, where n is 1-20 or (AK)n, where n is 1-20 or (LK)n, where n is 1-20 or (GA)n, where n is 1-20
CLPCLPAASCXXXXXXXXXXXXXXXXXXXXXXXXXXXXXXXXXXXXXXXX

SEQ ID NO: 544 - protein, 50 aa, synthetic construct
  VARIANT 11..50: note = This region may encompass one of the following sequences: (GQ)n, where n is 1-20 or (AK)n, where n is 1-20 or (LK)n, where n is 1-20 or (GA)n, where n is 1-20
CEPAICEPSCXXXXXXXXXXXXXXXXXXXXXXXXXXXXXXXXXXXXXXXX

SEQ ID NO: 545 - protein, 51 aa, synthetic construct
  VARIANT 12..51: note = This region may encompass one of the following sequences: (GQ)n, where n is 1-20 or (AK)n, where n is 1-20 or (LK)n, where n is 1-20 or (GA)n, where n is 1-20
CQCSCCKPYCSXXXXXXXXXXXXXXXXXXXXXXXXXXXXXXXXXXXXXXXX

SEQ ID NO: 546 - protein, 51 aa, synthetic construct
  VARIANT 12..51: note = This region may encompass one of the following sequences: (GQ)n, where n is 1-20 or (AK)n, where n is 1-20 or (LK)n, where n is 1-20 or (GA)n, where n is 1-20
FCGFPSCSTSCXXXXXXXXXXXXXXXXXXXXXXXXXXXXXXXXXXXXXXXX

SEQ ID NO: 547 - protein, 52 aa, synthetic construct
  VARIANT 13..52: note = This region may encompass one of the following sequences: (GQ)n, where n is 1-20 or (AK)n, where n is 1-20 or (LK)n, where n is 1-20 or (GA)n, where n is 1-20
CTPPSCCQLHHAXXXXXXXXXXXXXXXXXXXXXXXXXXXXXXXXXXXXXXXX

SEQ ID NO: 548 - protein, 50 aa, synthetic construct
  VARIANT 11..50: note = This region may encompass one of the following sequences: (GQ)n, where n is 1-20 or (AK)n, where n is 1-20 or (LK)n, where n is 1-20 or (GA)n, where n is 1-20
SCCAPVYCCKXXXXXXXXXXXXXXXXXXXXXXXXXXXXXXXXXXXXXXXX

SEQ ID NO: 549 - protein, 40 aa, synthetic construct
GGVCGPSPPCITTGAGAGSGAGAGSVPAVGVPAVGVPAVG

SEQ ID NO: 550 - protein, 82 aa, synthetic construct
GGVCGPSPPCITTRGAGAGSGAGAGSGAGAGSVPAVGVPAVGVPAVGVPAVGVPAVGVPAVGVPAVGVPAVGVPAVGVPAVG

SEQ ID NO: 551 - protein, 456 aa, synthetic construct; identical to SEQ ID NO: 108

SEQ ID NO: 552 - protein, 5 aa, synthetic construct
YGGFL

SEQ ID NO: 553 - protein, 4 aa, synthetic construct
YPWF

SEQ ID NO: 554 - protein, 5 aa, synthetic construct
YGGFM

SEQ ID NO: 555 - protein, 4 aa, synthetic construct
YPFF

SEQ ID NO: 556 - protein, 6 aa, synthetic construct
EEMQRR

SEQ ID NO: 557 - protein, 14 aa, synthetic construct
MGWCTASVPPQCYG

SEQ ID NO: 558 - protein, 18 aa, synthetic construct
ATAKAWLKGIGAGAGAGA

SEQ ID NO: 559 - protein, 14 aa, synthetic construct
RRQMEEGAGAGAGA

SEQ ID NO: 560 - protein, 23 aa, synthetic construct
GGVCGPSPPCITTATAKAWLKGI

SEQ ID NO: 561 - protein, 30 aa, synthetic construct
GGVCGPSPPCITTGAGAGAGATAKAWLKGI

SEQ ID NO: 562 - protein, 23 aa, synthetic construct
ATAKAWLKGIGGVCGPSPPCITT

SEQ ID NO: 563 - protein, 30 aa, synthetic construct
ATAKAWLKGIAGAGAGAGGVCGPSPPCITT

SEQ ID NO: 564 - protein, 29 aa, synthetic construct
GGVCGPSPPCITTATAKAWLKGIRRQMEE

SEQ ID NO: 565 - protein, 29 aa, synthetic construct
RRQMEEATAKAWLKGIGGVCGPSPPCITT

SEQ ID NO: 566 - protein, 19 aa, synthetic construct
GGVCGPSPPCITTRRQMEE

SEQ ID NO: 567 - protein, 26 aa, synthetic construct
GVCGPSPPCITTGAGAGAGARRQMEE

SEQ ID NO: 568 - protein, 27 aa, synthetic construct
RRQMEEGAGAGAGAGGVCGPSPPCITT

SEQ ID NO: 569 - protein, 24 aa, synthetic construct
ATAKAWLKGIMGWCTASVPPQCYG

SEQ ID NO: 570 - protein, 20 aa, synthetic construct
RRQMEEMGWCTASVPPQCYG

SEQ ID NO: 571 - protein, 11 aa, synthetic construct
YGRKKRRQRRR

SEQ ID NO: 572 - protein, 43 aa, synthetic construct
GGVCGPSPPCITTGTCYINDDEGCTKRCQGIYIYRREAVMGHC

SEQ ID NO: 573 - protein, 38 aa, synthetic construct
GGVCGPSPPCITTRCAERCSEASIQDRCLKYCGICCEK

SEQ ID NO: 574 - protein, 38 aa, synthetic construct
GGVCGPSPPCITTGTYGNKDECPCYRDMKNSKGKGKCP

SEQ ID NO: 575 - protein, 13 aa, synthetic construct
GRKKRRQRRRPPQ

SEQ ID NO: 576 - protein, 16 aa, synthetic construct
RQIKIWFQNRRMKWKK

SEQ ID NO: 577 - protein, 13 aa, synthetic construct
RIMRILRILKLAR

SEQ ID NO: 578 - protein, 19 aa, synthetic construct
LLIILRRRRIRKQAHAHSK

SEQ ID NO: 579 - protein, 24 aa, synthetic construct
GVCGPSPPCITTDRDDQAAWFSQY

SEQ ID NO: 580 - protein, 96 aa, synthetic construct
MVYYPNPCSPYPCRNGGTCKKRGLYSYKCYCRKGYTGKNCQYNACFPNPCLNGGTCGYVYGYPYYKCSCPYGYYGKQCQLKKYGGVCGPSPPCITT

SEQ ID NO: 581 - protein, 62 aa, synthetic construct
GGVCGPSPPCITTERSRSSDGKSSSQVNRSRHENTSQVPLQESRTRKRRGSRVSQDRDSEGH

SEQ ID NO: 582 - protein, 65 aa, synthetic construct
GGVCGPSPPCITTDGTRHSGSRHHEASSQADSSRHSQVGQGQSSGPRTSRNQGSSVSQDSDSQGH

SEQ ID NO: 583 - protein, 114 aa, synthetic construct
ERSRSSDGKSSSQVNRSRHENTSQVPLQESRTRKRRGSRVSQDRDSEGHGGVCGPSPPCITTDGTRHSGSRHHEASSQADSSRHSQVGQGQSSGPRTSRNQGSSVSQDSDSQGH

SEQ ID NO: 584 - protein, 27 aa, synthetic construct
GGVCGPSPPCITTGAGAGAGARRQMEE

SEQ ID NO: 585 - protein, 19 aa, synthetic construct
RRQMEEGGVCGPSPPCITT

SEQ ID NO: 586 - protein, 32 aa, synthetic construct
RRQMEEGGVCGPSPPCITTGRKKRRQRRRPPQ

SEQ ID NO: 587 - protein, 32 aa, synthetic construct
GRKKRRQRRRPPQGGVCGPSPPCITTRRQMEE

SEQ ID NO: 588 - protein, 20 aa, synthetic construct
LKLKLKLKLKLKLKLKLKLK

SEQ ID NO: 589 - protein, 20 aa, synthetic construct
LELELELELELELELELELE

SEQ ID NO: 590 - protein, 10 aa, synthetic construct
RKKNPNCRRH